European Patent Application EP 4 570 906 A1, published June 18, 2025. Title: METHOD FOR EPITOPE EDITING TARGET AND USE. Applicant: Epigenic Therapeutics, Inc. The sequence listing filed with the application follows.

SEQUENCE LISTING (113 sequences)

SEQ ID NO: 1 - RNA, 20 nt, synthetic construct
  modified_base 2: mod_base = OTHER; note = thymine
  modified_base 15: mod_base = OTHER; note = thymine
  misc_feature 1..20: note = hLPA-1
  source 1..20: mol_type = other RNA
gtagcgacacaacctcggga

SEQ ID NO: 2 - RNA, 20 nt, synthetic construct
  modified_base 10: mod_base = OTHER; note = thymine
  modified_base 19: mod_base = OTHER; note = thymine
  misc_feature 1..20: note = hLPA-2
  source 1..20: mol_type = other RNA
aaggagacataaaggcaatg

SEQ ID NO: 3 - RNA, 20 nt, synthetic construct
  modified_base 8: mod_base = OTHER; note = thymine
  modified_base 10: mod_base = OTHER; note = thymine
  modified_base 14: mod_base = OTHER; note = thymine
  modified_base 18: mod_base = OTHER; note = thymine
  misc_feature 1..20: note = hLPA-3
  source 1..20: mol_type = other RNA
aaaagagtgtgcctacatga

SEQ ID NO: 4 - RNA, 20 nt, synthetic construct
  modified_base 9: mod_base = OTHER; note = thymine
  modified_base 15: mod_base = OTHER; note = thymine
  modified_base 18: mod_base = OTHER; note = thymine
  modified_base 20: mod_base = OTHER; note = thymine
  misc_feature 1..20: note = hLPA-4
  source 1..20: mol_type = other RNA
agccagactggccatcatgt

SEQ ID NO: 5 - RNA, 20 nt, synthetic construct
  modified_base 7: mod_base = OTHER; note = thymine
  modified_base 10: mod_base = OTHER; note = thymine
  modified_base 12: mod_base = OTHER; note = thymine
  misc_feature 1..20: note = hLPA-5
  source 1..20: mol_type = other RNA
aggcagtgctgtacgaggag

SEQ ID NO: 6 - RNA, 20 nt, synthetic construct
  modified_base 4: mod_base = OTHER; note = thymine
  modified_base 8: mod_base = OTHER; note = thymine
  modified_base 13: mod_base = OTHER; note = thymine
  modified_base 15..16: mod_base = OTHER; note = thymine
  modified_base 20: mod_base = OTHER; note = thymine
  misc_feature 1..20: note = hLPA-6
  source 1..20: mol_type = other RNA
ggatggctaagctcttcgct

SEQ ID NO: 7 - RNA, 20 nt, synthetic construct
  modified_base 3: mod_base = OTHER; note = thymine
  modified_base 5..6: mod_base = OTHER; note = thymine
  modified_base 14..15: mod_base = OTHER; note = thymine
  misc_feature 1..20: note = hLPA-7
  source 1..20: mol_type = other RNA
cctgttggaaagcttgaggg

SEQ ID NO: 8 - RNA, 20 nt, synthetic construct
  modified_base 12: mod_base = OTHER; note = thymine
  modified_base 15: mod_base = OTHER; note = thymine
  modified_base 17: mod_base = OTHER; note = thymine
  misc_feature 1..20: note = hLPA-8
  source 1..20: mol_type = other RNA
ccaacaggcagtgctgtacg

SEQ ID NO: 9 - RNA, 20 nt, synthetic construct
  modified_base 2: mod_base = OTHER; note = thymine
  modified_base 6: mod_base = OTHER; note = thymine
  modified_base 19: mod_base = OTHER; note = thymine
  misc_feature 1..20: note = hLPA-9
  source 1..20: mol_type = other RNA
ctgggtagcgacacaacctc

SEQ ID NO: 10 - RNA, 20 nt, synthetic construct
  modified_base 2: mod_base = OTHER; note = thymine
  modified_base 7: mod_base = OTHER; note = thymine
  modified_base 9: mod_base = OTHER; note = thymine
  modified_base 13: mod_base = OTHER; note = thymine
  modified_base 17: mod_base = OTHER; note = thymine
  modified_base 20: mod_base = OTHER; note = thymine
  misc_feature 1..20: note = hLPA-10
  source 1..20: mol_type = other RNA
gtgcaatgtcaatagatgct

SEQ ID NO: 11 - RNA, 20 nt, synthetic construct
  modified_base 4: mod_base = OTHER; note = thymine
  modified_base 6: mod_base = OTHER; note = thymine
  modified_base 15: mod_base = OTHER; note = thymine
  misc_feature 1..20: note = hLPA-11
  source 1..20: mol_type = other RNA
caatgtggagcagctgaggg

SEQ ID NO: 12 - RNA, 20 nt, synthetic construct
  modified_base 7: mod_base = OTHER; note = thymine
  modified_base 13: mod_base = OTHER; note = thymine
  modified_base 15..16: mod_base = OTHER; note = thymine
  misc_feature 1..20: note = hLPA-12
  source 1..20: mol_type = other RNA
gcaccgtgacagtcttcacg

SEQ ID NO: 13 - RNA, 20 nt, synthetic construct
  modified_base 3: mod_base = OTHER; note = thymine
  modified_base 8: mod_base = OTHER; note = thymine
  modified_base 10: mod_base = OTHER; note = thymine
  modified_base 14: mod_base = OTHER; note = thymine
  modified_base 18: mod_base = OTHER; note = thymine
  misc_feature 1..20: note = hLPA-13
  source 1..20: mol_type = other RNA
agtgcaatgtcaatagatgc

SEQ ID NO: 14 - RNA, 20 nt, synthetic construct
  modified_base 7: mod_base = OTHER; note = thymine
  modified_base 9: mod_base = OTHER; note = thymine
  modified_base 18: mod_base = OTHER; note = thymine
  misc_feature 1..20: note = hLPA-14
  source 1..20: mol_type = other RNA
aggcaatgtggagcagctga

SEQ ID NO: 15 - RNA, 20 nt, synthetic construct
  modified_base 1..3: mod_base = OTHER; note = thymine
  modified_base 9: mod_base = OTHER; note = thymine
  modified_base 16: mod_base = OTHER; note = thymine
  modified_base 18: mod_base = OTHER; note = thymine
  misc_feature 1..20: note = hLPA-15
  source 1..20: mol_type = other RNA
tttccccgtgaagactgtca

SEQ ID NO: 16 - RNA, 20 nt, synthetic construct
  modified_base 8: mod_base = OTHER; note = thymine
  modified_base 10: mod_base = OTHER; note = thymine
  modified_base 19: mod_base = OTHER; note = thymine
  misc_feature 1..20: note = hLPA-16
  source 1..20: mol_type = other RNA
aaggcaatgtggagcagctg

SEQ ID NO: 17 - RNA, 20 nt, synthetic construct
  modified_base 5: mod_base = OTHER; note = thymine
  modified_base 7: mod_base = OTHER; note = thymine
  modified_base 16: mod_base = OTHER; note = thymine
  misc_feature 1..20: note = hLPA-17
  source 1..20: mol_type = other RNA
gcaatgtggagcagctgagg

SEQ ID NO: 18 - RNA, 20 nt, synthetic construct
  modified_base 6: mod_base = OTHER; note = thymine
  modified_base 8: mod_base = OTHER; note = thymine
  modified_base 17: mod_base = OTHER; note = thymine
  misc_feature 1..20: note = hLPA-18
  source 1..20: mol_type = other RNA
ggcaatgtggagcagctgag

SEQ ID NO: 19 - RNA, 20 nt, synthetic construct
  modified_base 1..3: mod_base = OTHER; note = thymine
  modified_base 10: mod_base = OTHER; note = thymine
  modified_base 13: mod_base = OTHER; note = thymine
  misc_feature 1..20: note = hLPA-19
  source 1..20: mol_type = other RNA
tttgaaccctgctgagccag

SEQ ID NO: 20 - RNA, 20 nt, synthetic construct
  modified_base 5: mod_base = OTHER; note = thymine
  modified_base 11: mod_base = OTHER; note = thymine
  modified_base 15: mod_base = OTHER; note = thymine
  misc_feature 1..20: note = hLPA-20
  source 1..20: mol_type = other RNA
cccatgccactggctcagca

SEQ ID NO: 21 - RNA, 20 nt, synthetic construct
  modified_base 1: mod_base = OTHER; note = thymine
  modified_base 3: mod_base = OTHER; note = thymine
  modified_base 7: mod_base = OTHER; note = thymine
  modified_base 11: mod_base = OTHER; note = thymine
  modified_base 14: mod_base = OTHER; note = thymine
  misc_feature 1..20: note = hLPA-21
  source 1..20: mol_type = other RNA
tgtcaatagatgctgggaag

SEQ ID NO: 22 - RNA, 20 nt, synthetic construct
  modified_base 9: mod_base = OTHER; note = thymine
  modified_base 15: mod_base = OTHER; note = thymine
  modified_base 17..18: mod_base = OTHER; note = thymine
  misc_feature 1..20: note = hLPA-22
  source 1..20: mol_type = other RNA
cagcaccgtgacagtcttca

SEQ ID NO: 23 - RNA, 20 nt, synthetic construct
  modified_base 1: mod_base = OTHER; note = thymine
  modified_base 3: mod_base = OTHER; note = thymine
  modified_base 5: mod_base = OTHER; note = thymine
  modified_base 7..11: mod_base = OTHER; note = thymine
  modified_base 14: mod_base = OTHER; note = thymine
  modified_base 18..19: mod_base = OTHER; note = thymine
  misc_feature 1..20: note = hLPA-23
  source 1..20: mol_type = other RNA
tatgtatttttactacattg

SEQ ID NO: 24 - RNA, 20 nt, synthetic construct
  modified_base 1: mod_base = OTHER; note = thymine
  modified_base 4: mod_base = OTHER; note = thymine
  modified_base 10: mod_base = OTHER; note = thymine
  modified_base 14: mod_base = OTHER; note = thymine
  modified_base 16: mod_base = OTHER; note = thymine
  misc_feature 1..20: note = hLPA-24
  source 1..20: mol_type = other RNA
tagtaaaaatacatatgcca

SEQ ID NO: 25 - RNA, 20 nt, synthetic construct
  modified_base 2: mod_base = OTHER; note = thymine
  modified_base 4: mod_base = OTHER; note = thymine
  modified_base 8: mod_base = OTHER; note = thymine
  modified_base 15: mod_base = OTHER; note = thymine
  modified_base 17: mod_base = OTHER; note = thymine
  modified_base 20: mod_base = OTHER; note = thymine
  misc_feature 1..20: note = hLPA-25
  source 1..20: mol_type = other RNA
atgtaagtcaacaatgtcct

SEQ ID NO: 26 - RNA, 20 nt, synthetic construct
  modified_base 1..3: mod_base = OTHER; note = thymine
  modified_base 5: mod_base = OTHER; note = thymine
  modified_base 11: mod_base = OTHER; note = thymine
  modified_base 13: mod_base = OTHER; note = thymine
  modified_base 15: mod_base = OTHER; note = thymine
  modified_base 17..18: mod_base = OTHER; note = thymine
  misc_feature 1..20: note = hLPA-26
  source 1..20: mol_type = other RNA
tttataagactctatattca

SEQ ID NO: 27 - RNA, 20 nt, synthetic construct
  modified_base 9: mod_base = OTHER; note = thymine
  misc_feature 1..20: note = hLPA-27
  source 1..20: mol_type = other RNA
ggagcagctgaggggggaaa

SEQ ID NO: 28 - RNA, 20 nt, synthetic construct
  modified_base 5: mod_base = OTHER; note = thymine
  modified_base 8: mod_base = OTHER; note = thymine
  modified_base 16: mod_base = OTHER; note = thymine
  misc_feature 1..20: note = hLPA-28
  source 1..20: mol_type = other RNA
accctgctgagccagtggca

SEQ ID NO: 29 - RNA, 20 nt, synthetic construct
  modified_base 2: mod_base = OTHER; note = thymine
  modified_base 6..7: mod_base = OTHER; note = thymine
  modified_base 13: mod_base = OTHER; note = thymine
  misc_feature 1..20: note = hLPA-29
  source 1..20: mol_type = other RNA
atgaattgcacataaagcca

SEQ ID NO: 30 - RNA, 20 nt, synthetic construct
  modified_base 8: mod_base = OTHER; note = thymine
  modified_base 18: mod_base = OTHER; note = thymine
  misc_feature 1..20: note = hLPA-30
  source 1..20: mol_type = other RNA
gaaggagtaaggagacataa

SEQ ID NO: 31 - RNA, 20 nt, synthetic construct
  modified_base 8: mod_base = OTHER; note = thymine
  modified_base 14: mod_base = OTHER; note = thymine
  modified_base 16..17: mod_base = OTHER; note = thymine
  misc_feature 1..20: note = hLPA-31
  source 1..20: mol_type = other RNA
agcaccgtgacagtcttcac

SEQ ID NO: 32 - RNA, 20 nt, synthetic construct
  modified_base 3: mod_base = OTHER; note = thymine
  modified_base 5: mod_base = OTHER; note = thymine
  modified_base 12..15: mod_base = OTHER; note = thymine
  modified_base 20: mod_base = OTHER; note = thymine
  misc_feature 1..20: note = hLPA-32
  source 1..20: mol_type = other RNA
catatacaagattttgaact

SEQ ID NO: 33 - RNA, 20 nt, synthetic construct
  modified_base 2: mod_base = OTHER; note = thymine
  modified_base 4: mod_base = OTHER; note = thymine
  modified_base 15: mod_base = OTHER; note = thymine
  misc_feature 1..20: note = hLPA-33
  source 1..20: mol_type = other RNA
ctctcagagacccatgccac

SEQ ID NO: 34 - RNA, 20 nt, synthetic construct
  modified_base 3: mod_base = OTHER; note = thymine
  modified_base 10: mod_base = OTHER; note = thymine
  modified_base 12: mod_base = OTHER; note = thymine
  modified_base 15: mod_base = OTHER; note = thymine
  modified_base 20: mod_base = OTHER; note = thymine
  misc_feature 1..20: note = hLPA-34
  source 1..20: mol_type = other RNA
agtcaacaatgtcctgggat

SEQ ID NO: 35 - RNA, 20 nt, synthetic construct
  modified_base 6: mod_base = OTHER; note = thymine
  modified_base 13: mod_base = OTHER; note = thymine
  misc_feature 1..20: note = hLPA-35
  source 1..20: mol_type = other RNA
caaaatggaacataaggaag

SEQ ID NO: 36 - RNA, 20 nt, synthetic construct
  modified_base 3: mod_base = OTHER; note = thymine
  modified_base 5: mod_base = OTHER; note = thymine
  modified_base 9: mod_base = OTHER; note = thymine
  modified_base 16: mod_base = OTHER; note = thymine
  modified_base 18: mod_base = OTHER; note = thymine
  misc_feature 1..20: note = hLPA-36
  source 1..20: mol_type = other RNA
catgtaagtcaacaatgtcc

SEQ ID NO: 37 - RNA, 20 nt, synthetic construct
  modified_base 7: mod_base = OTHER; note = thymine
  modified_base 9: mod_base = OTHER; note = thymine
  modified_base 11: mod_base = OTHER; note = thymine
  modified_base 17: mod_base = OTHER; note = thymine
  misc_feature 1..20: note = hLPA-37
  source 1..20: mol_type = other RNA
agaaagtgtgtcccaatccc

SEQ ID NO: 38 - RNA, 20 nt, synthetic construct
  modified_base 2: mod_base = OTHER; note = thymine
  modified_base 4: mod_base = OTHER; note = thymine
  modified_base 6..10: mod_base = OTHER; note = thymine
  modified_base 13: mod_base = OTHER; note = thymine
  modified_base 17..18: mod_base = OTHER; note = thymine
  modified_base 20: mod_base = OTHER; note = thymine
  misc_feature 1..20: note = hLPA-38
  source 1..20: mol_type = other RNA
atgtatttttactacattgt

SEQ ID NO: 39 - RNA, 20 nt, synthetic construct
  modified_base 4: mod_base = OTHER; note = thymine
  modified_base 12: mod_base = OTHER; note = thymine
  modified_base 19: mod_base = OTHER; note = thymine
  misc_feature 1..20: note = hLPA-39
  source 1..20: mol_type = other RNA
cagtcccaaaatggaacata

SEQ ID NO: 40 - RNA, 20 nt, synthetic construct
  modified_base 2: mod_base = OTHER; note = thymine
  modified_base 9: mod_base = OTHER; note = thymine
  modified_base 11: mod_base = OTHER; note = thymine
  modified_base 14: mod_base = OTHER; note = thymine
  modified_base 19..20: mod_base = OTHER; note = thymine
  misc_feature 1..20: note = hLPA-40
  source 1..20: mol_type = other RNA
gtcaacaatgtcctgggatt

SEQ ID NO: 41 - RNA, 20 nt, synthetic construct
  modified_base 6: mod_base = OTHER; note = thymine
  modified_base 12: mod_base = OTHER; note = thymine
  modified_base 16: mod_base = OTHER; note = thymine
  misc_feature 1..20: note = hLPA-41
  source 1..20: mol_type = other RNA
acccatgccactggctcagc

SEQ ID NO: 42 - RNA, 20 nt, synthetic construct
  modified_base 4: mod_base = OTHER; note = thymine
  modified_base 7: mod_base = OTHER; note = thymine
  modified_base 15: mod_base = OTHER; note = thymine
  modified_base 20: mod_base = OTHER; note = thymine
  misc_feature 1..20: note = hLPA-42
  source 1..20: mol_type = other RNA
ccctgctgagccagtggcat

SEQ ID NO: 43 - RNA, 20 nt, synthetic construct
  modified_base 1: mod_base = OTHER; note = thymine
  modified_base 4..6: mod_base = OTHER; note = thymine
  modified_base 10: mod_base = OTHER; note = thymine
  modified_base 12: mod_base = OTHER; note = thymine
  modified_base 14: mod_base = OTHER; note = thymine
  modified_base 17..19: mod_base = OTHER; note = thymine
  misc_feature 1..20: note = hLPA-43
  source 1..20: mol_type = other RNA
taatttgactatctggtttg

SEQ ID NO: 44 - RNA, 20 nt, synthetic construct
  modified_base 1: mod_base = OTHER; note = thymine
  modified_base 4: mod_base = OTHER; note = thymine
  modified_base 6: mod_base = OTHER; note = thymine
  modified_base 13..16: mod_base = OTHER; note = thymine
  misc_feature 1..20: note = hLPA-44
  source 1..20: mol_type = other RNA
tcatatacaagattttgaac

SEQ ID NO: 45 - RNA, 20 nt, synthetic construct
  modified_base 3..5: mod_base = OTHER; note = thymine
  modified_base 9: mod_base = OTHER; note = thymine
  modified_base 11: mod_base = OTHER; note = thymine
  modified_base 13: mod_base = OTHER; note = thymine
  modified_base 16..18: mod_base = OTHER; note = thymine
  modified_base 20: mod_base = OTHER; note = thymine
  misc_feature 1..20: note = hLPA-45
  source 1..20: mol_type = other RNA
aatttgactatctggtttgt

SEQ ID NO: 46 - RNA, 20 nt, synthetic construct
  modified_base 7..9: mod_base = OTHER; note = thymine
  modified_base 11: mod_base = OTHER; note = thymine
  modified_base 18: mod_base = OTHER; note = thymine
  misc_feature 1..20: note = hLPA-46
  source 1..20: mol_type = other RNA
acacactttctgggcactgc

SEQ ID NO: 47 - RNA, 20 nt, synthetic construct
  modified_base 3: mod_base = OTHER; note = thymine
  modified_base 6: mod_base = OTHER; note = thymine
  modified_base 13: mod_base = OTHER; note = thymine
  misc_feature 1..20: note = hLPA-47
  source 1..20: mol_type = other RNA
actgctggccagtcccaaaa

SEQ ID NO: 48 - RNA, 20 nt, synthetic construct
  modified_base 2..3: mod_base = OTHER; note = thymine
  modified_base 5..8: mod_base = OTHER; note = thymine
  modified_base 10..12: mod_base = OTHER; note = thymine
  modified_base 14: mod_base = OTHER; note = thymine
  modified_base 19: mod_base = OTHER; note = thymine
  misc_feature 1..20: note = hLPA-48
  source 1..20: mol_type = other RNA
cttcttttatttctgaaatc

SEQ ID NO: 49 - RNA, 20 nt, synthetic construct
  modified_base 2..3: mod_base = OTHER; note = thymine
  modified_base 5: mod_base = OTHER; note = thymine
  modified_base 7..8: mod_base = OTHER; note = thymine
  modified_base 12..15: mod_base = OTHER; note = thymine
  misc_feature 1..20: note = hLPA-49
  source 1..20: mol_type = other RNA
cttatgttccattttgggac

SEQ ID NO: 50 - RNA, 20 nt, synthetic construct
  modified_base 5..6: mod_base = OTHER; note = thymine
  modified_base 16..18: mod_base = OTHER; note = thymine
  modified_base 20: mod_base = OTHER; note = thymine
  misc_feature 1..20: note = hLPA-50
  source 1..20: mol_type = other RNA
gggattgggacacactttct

SEQ ID NO: 51 - DNA, 1000 bp, synthetic construct
  misc_feature 1..1000: note = hLPA subregion
  source 1..1000: mol_type = other DNA
actaagacctgaaagggttgtgtctatcagctgcacccctgggtagcgacacaacctcgggaaggcctcagccccctcctcgtacagcactgcctgttggaaagcttgagggaggctatggatgtgcagcacttggcagagggtctggtcatggaagttaccagcaaatatgagctacttttatgattttattttatccaaaagaaagagaatgaaagaagaggggaggaaacaagactaatcaggaaagatgaaggtctaggggtgagggaaggagtaaggagacataaaggcaatgtggagcagctgaggggggaaatggctttcaccacttcccagcatctattgacattgcactctcaaatattttataagactctatattcaaggtaatgtttgaaccctgctgagccagtggcatgggtctctgagagaatcattaacttaatttgactatctggtttgtgggtgcgtttactctcatgtaagtcaacaatgtcctgggattgggacacactttctgggcactgctggccagtcccaaaatggaacataaggaagtggttcttctacttcttttatttctgaaatcaggtaagacatagtttttttaaattataagaattattttttctcccacaatgtagtaaaaatacatatgccatggctttatgtgcaattcatttaatttttgattcatgaaattcccagttcaaaatcttgtatatgattgaaaaattcttaaaaaaataagtttaatttccccgtgaagactgtcacggtgctggaatgaatgggcagaaaaaataatggttgatttttctaatctaaaagagtgtgcctacatgatggccagtctggctgaaaaataaatagccattgtagctaactatgcaaaggatggctaagctcttcgcttggttctcagtttcattaatttatatcatctctgttcaggtgccatgctcccctcactagcaagttgaaacaatgaaataac

SEQ ID NO: 52 - DNA, 80 bp, synthetic construct
  misc_feature 1..80: note = hLPA-1 target
  source 1..80: mol_type = other DNA
aagggttgtgtctatcagctgcacccctgggtagcgacacaacctcgggaaggcctcagccccctcctcgtacagcactg

SEQ ID NO: 53 - DNA, 80 bp, synthetic construct
  misc_feature 1..80: note = hLPA-2 target
  source 1..80: mol_type = other DNA
agatgaaggtctaggggtgagggaaggagtaaggagacataaaggcaatgtggagcagctgaggggggaaatggctttca

SEQ ID NO: 54 - DNA, 80 bp, synthetic construct
  misc_feature 1..80: note = hLPA-3 target
  source 1..80: mol_type = other DNA
agaaaaaataatggttgatttttctaatctaaaagagtgtgcctacatgatggccagtctggctgaaaaataaatagcca

SEQ ID NO: 55 - DNA, 80 bp, synthetic construct
  misc_feature 1..80: note = hLPA-4 target
  source 1..80: mol_type = other DNA
atagttagctacaatggctatttatttttcagccagactggccatcatgtaggcacactcttttagattagaaaaatcaa

SEQ ID NO: 56 - DNA, 80 bp, synthetic construct
  misc_feature 1..80: note = hLPA-5 target
  source 1..80: mol_type = other DNA
acatccatagcctccctcaagctttccaacaggcagtgctgtacgaggagggggctgaggccttcccgaggttgtgtcgc

SEQ ID NO: 57 - DNA, 80 bp, synthetic construct
  misc_feature 1..80: note = hLPA-6 target
  source 1..80: mol_type = other DNA
ataaatagccattgtagctaactatgcaaaggatggctaagctcttcgcttggttctcagtttcattaatttatatcatc

SEQ ID NO: 58 - DNA, 80 bp, synthetic construct
  misc_feature 1..80: note = hLPA-7 target
  source 1..80: mol_type = other DNA
aggcctcagccccctcctcgtacagcactgcctgttggaaagcttgagggaggctatggatgtgcagcacttggcagagg

SEQ ID NO: 59 - DNA, 80 bp, synthetic construct
  misc_feature 1..80: note = hLPA-8 target
  source 1..80: mol_type = other DNA
gctgcacatccatagcctccctcaagctttccaacaggcagtgctgtacgaggagggggctgaggccttcccgaggttgt

SEQ ID NO: 60 - DNA, 80 bp, synthetic construct
  misc_feature 1..80: note = hLPA-9 target
  source 1..80: mol_type = other DNA
ctgaaagggttgtgtctatcagctgcacccctgggtagcgacacaacctcgggaaggcctcagccccctcctcgtacagc

SEQ ID NO: 61 - DNA, 80 bp, synthetic construct
  misc_feature 1..80: note = hLPA-10 target
  source 1..80: mol_type = other DNA
tgaatatagagtcttataaaatatttgagagtgcaatgtcaatagatgctgggaagtggtgaaagccatttcccccctca

SEQ ID NO: 62 - DNA, 80 bp, synthetic construct
  misc_feature 1..80: note = hLPA-11 target
  source 1..80: mol_type = other DNA
ggtgagggaaggagtaaggagacataaaggcaatgtggagcagctgaggggggaaatggctttcaccacttcccagcatc

SEQ ID NO: 63 - DNA, 80 bp, synthetic construct
  misc_feature 1..80: note = hLPA-12 target
  source 1..80: mol_type = other DNA
aaccattattttttctgcccattcattccagcaccgtgacagtcttcacggggaaattaaacttatttttttaagaattt

SEQ ID NO: 64 - DNA, 80 bp, synthetic construct
  misc_feature 1..80: note = hLPA-13 target
  source 1..80: mol_type = other DNA
ttgaatatagagtcttataaaatatttgagagtgcaatgtcaatagatgctgggaagtggtgaaagccatttcccccctc

SEQ ID NO: 65 - DNA, 80 bp, synthetic construct
  misc_feature 1..80: note = hLPA-14 target
  source 1..80: mol_type = other DNA
aggggtgagggaaggagtaaggagacataaaggcaatgtggagcagctgaggggggaaatggctttcaccacttcccagc

SEQ ID NO: 66 - DNA, 80 bp, synthetic construct
  misc_feature 1..80: note = hLPA-15 target
  source 1..80: mol_type = other DNA
attgaaaaattcttaaaaaaataagtttaatttccccgtgaagactgtcacggtgctggaatgaatgggcagaaaaaata

SEQ ID NO: 67 - DNA, 80 bp, synthetic construct
  misc_feature 1..80: note = hLPA-16 target
  source 1..80: mol_type = other DNA
taggggtgagggaaggagtaaggagacataaaggcaatgtggagcagctgaggggggaaatggctttcaccacttcccag

SEQ ID NO: 68 - DNA, 80 bp, synthetic construct
  misc_feature 1..80: note = hLPA-17 target
  source 1..80: mol_type = other DNA
gggtgagggaaggagtaaggagacataaaggcaatgtggagcagctgaggggggaaatggctttcaccacttcccagcat

SEQ ID NO: 69 - DNA, 80 bp, synthetic construct
  misc_feature 1..80: note = hLPA-18 target
  source 1..80: mol_type = other DNA
ggggtgagggaaggagtaaggagacataaaggcaatgtggagcagctgaggggggaaatggctttcaccacttcccagca

SEQ ID NO: 70 - DNA, 80 bp, synthetic construct
  misc_feature 1..80: note = hLPA-19 target
  source 1..80: mol_type = other DNA
attttataagactctatattcaaggtaatgtttgaaccctgctgagccagtggcatgggtctctgagagaatcattaact

SEQ ID NO: 71 - DNA, 80 bp, synthetic construct
  misc_feature 1..80: note = hLPA-20 target
  source 1..80: mol_type = other DNA
gtcaaattaagttaatgattctctcagagacccatgccactggctcagcagggttcaaacattaccttgaatatagagtc

SEQ ID NO: 72 - DNA, 80 bp, synthetic construct
  misc_feature 1..80: note = hLPA-21 target
  source 1..80: mol_type = other DNA
tagagtcttataaaatatttgagagtgcaatgtcaatagatgctgggaagtggtgaaagccatttcccccctcagctgct

SEQ ID NO: 73 - DNA, 80 bp, synthetic construct
  misc_feature 1..80: note = hLPA-22 target
  source 1..80: mol_type = other DNA
tcaaccattattttttctgcccattcattccagcaccgtgacagtcttcacggggaaattaaacttatttttttaagaat

SEQ ID NO: 74 - DNA, 80 bp, synthetic construct
  misc_feature 1..80: note = hLPA-23 target
  source 1..80: mol_type = other DNA
attaaatgaattgcacataaagccatggcatatgtatttttactacattgtgggagaaaaaataattcttataatttaaa

SEQ ID NO: 75 - DNA, 80 bp, synthetic construct
  misc_feature 1..80: note = hLPA-24 target
  source 1..80: mol_type = other DNA
attataagaattattttttctcccacaatgtagtaaaaatacatatgccatggctttatgtgcaattcatttaatttttg

SEQ ID NO: 76 - DNA, 80 bp, synthetic construct
  misc_feature 1..80: note = hLPA-25 target
  source 1..80: mol_type = other DNA
actatctggtttgtgggtgcgtttactctcatgtaagtcaacaatgtcctgggattgggacacactttctgggcactgct

SEQ ID NO: 77 - DNA, 80 bp, synthetic construct
  misc_feature 1..80: note = hLPA-26 target
  source 1..80: mol_type = other DNA
agcatctattgacattgcactctcaaatattttataagactctatattcaaggtaatgtttgaaccctgctgagccagtg

SEQ ID NO: 78 - DNA, 80 bp, synthetic construct
  misc_feature 1..80: note = hLPA-27 target
  source 1..80: mol_type = other DNA
ggaaggagtaaggagacataaaggcaatgtggagcagctgaggggggaaatggctttcaccacttcccagcatctattga

SEQ ID NO: 79 - DNA, 80 bp, synthetic construct
  misc_feature 1..80: note = hLPA-28 target
  source 1..80: mol_type = other DNA
ataagactctatattcaaggtaatgtttgaaccctgctgagccagtggcatgggtctctgagagaatcattaacttaatt

SEQ ID NO: 80 - DNA, 80 bp, synthetic construct
  misc_feature 1..80: note = hLPA-29 target
  source 1..80: mol_type = other DNA
gaactgggaatttcatgaatcaaaaattaaatgaattgcacataaagccatggcatatgtatttttactacattgtggga

SEQ ID NO: 81 - DNA, 80 bp, synthetic construct
  misc_feature 1..80: note = hLPA-30 target
  source 1..80: mol_type = other DNA
atcaggaaagatgaaggtctaggggtgagggaaggagtaaggagacataaaggcaatgtggagcagctgaggggggaaat

SEQ ID NO: 82 - DNA, 80 bp, synthetic construct
  misc_feature 1..80: note = hLPA-31 target
  source 1..80: mol_type = other DNA
caaccattattttttctgcccattcattccagcaccgtgacagtcttcacggggaaattaaacttatttttttaagaatt

SEQ ID NO: 83 - DNA, 80 bp, synthetic construct
  misc_feature 1..80: note = hLPA-32 target
  source 1..80: mol_type = other DNA
ttaaacttatttttttaagaatttttcaatcatatacaagattttgaactgggaatttcatgaatcaaaaattaaatgaa

SEQ ID NO: 84 - DNA, 80 bp, synthetic construct
  misc_feature 1..80: note = hLPA-33 target
  source 1..80: mol_type = other DNA
aaaccagatagtcaaattaagttaatgattctctcagagacccatgccactggctcagcagggttcaaacattaccttga

SEQ ID NO: 85 - DNA, 80 bp, synthetic construct
  misc_feature 1..80: note = hLPA-34 target
  source 1..80: mol_type = other DNA
ctggtttgtgggtgcgtttactctcatgtaagtcaacaatgtcctgggattgggacacactttctgggcactgctggcca

SEQ ID NO: 86 - DNA, 80 bp, synthetic construct
  misc_feature 1..80: note = hLPA-35 target
  source 1..80: mol_type = other DNA
acacactttctgggcactgctggccagtcccaaaatggaacataaggaagtggttcttctacttcttttatttctgaaat

SEQ ID NO: 87 - DNA, 80 bp, synthetic construct
  misc_feature 1..80: note = hLPA-36 target
  source 1..80: mol_type = other DNA
gactatctggtttgtgggtgcgtttactctcatgtaagtcaacaatgtcctgggattgggacacactttctgggcactgc

SEQ ID NO: 88 - DNA, 80 bp, synthetic construct
  misc_feature 1..80: note = hLPA-37 target
  source 1..80: mol_type = other DNA
gttccattttgggactggccagcagtgcccagaaagtgtgtcccaatcccaggacattgttgacttacatgagagtaaac

SEQ ID NO: 89 - DNA, 80 bp, synthetic construct
  misc_feature 1..80: note = hLPA-38 target
  source 1..80: mol_type = other DNA
ttaaatgaattgcacataaagccatggcatatgtatttttactacattgtgggagaaaaaataattcttataatttaaaa

SEQ ID NO: 90 - DNA, 80 bp, synthetic construct
  misc_feature 1..80: note = hLPA-39 target
  source 1..80: mol_type = other DNA
attgggacacactttctgggcactgctggccagtcccaaaatggaacataaggaagtggttcttctacttcttttatttc

SEQ ID NO: 91 - DNA, 80 bp, synthetic construct
  misc_feature 1..80: note = hLPA-40 target
  source 1..80: mol_type = other DNA
tggtttgtgggtgcgtttactctcatgtaagtcaacaatgtcctgggattgggacacactttctgggcactgctggccag

SEQ ID NO: 92 - DNA, 80 bp, synthetic construct
  misc_feature 1..80: note = hLPA-41 target
  source 1..80: mol_type = other DNA
agtcaaattaagttaatgattctctcagagacccatgccactggctcagcagggttcaaacattaccttgaatatagagt

SEQ ID NO: 93 - DNA, 80 bp, synthetic construct
  misc_feature 1..80: note = hLPA-42 target
  source 1..80: mol_type = other DNA
taagactctatattcaaggtaatgtttgaaccctgctgagccagtggcatgggtctctgagagaatcattaacttaattt

SEQ ID NO: 94 - DNA, 80 bp, synthetic construct
  misc_feature 1..80: note = hLPA-43 target
  source 1..80: mol_type = other DNA
tggcatgggtctctgagagaatcattaacttaatttgactatctggtttgtgggtgcgtttactctcatgtaagtcaaca

SEQ ID NO: 95 - DNA, 80 bp, synthetic construct
  misc_feature 1..80: note = hLPA-44 target
  source 1..80: mol_type = other DNA
attaaacttatttttttaagaatttttcaatcatatacaagattttgaactgggaatttcatgaatcaaaaattaaatga

SEQ ID NO: 96 - DNA, 80 bp, synthetic construct
  misc_feature 1..80: note = hLPA-45 target
  source 1..80: mol_type = other DNA
ggcatgggtctctgagagaatcattaacttaatttgactatctggtttgtgggtgcgtttactctcatgtaagtcaacaa

SEQ ID NO: 97 - DNA, 80 bp, synthetic construct
  misc_feature 1..80: note = hLPA-46 target
  source 1..80: mol_type = other DNA
catgtaagtcaacaatgtcctgggattgggacacactttctgggcactgctggccagtcccaaaatggaacataaggaag

SEQ ID NO: 98 - DNA, 80 bp, synthetic construct
  misc_feature 1..80: note = hLPA-47 target
  source 1..80: mol_type = other DNA
tgtcctgggattgggacacactttctgggcactgctggccagtcccaaaatggaacataaggaagtggttcttctacttc

SEQ ID NO: 99 - DNA, 80 bp, synthetic construct
  misc_feature 1..80: note = hLPA-48 target
  source 1..80: mol_type = other DNA
aaaatggaacataaggaagtggttcttctacttcttttatttctgaaatcaggtaagacatagtttttttaaattataag

SEQ ID NO: 100 - DNA, 80 bp, synthetic construct
  misc_feature 1..80: note = hLPA-49 target
  source 1..80: mol_type = other DNA
cagaaataaaagaagtagaagaaccacttccttatgttccattttgggactggccagcagtgcccagaaagtgtgtccca

SEQ ID NO: 101 - DNA, 80 bp, synthetic construct
  misc_feature 1..80: note = hLPA-50 target
  source 1..80: mol_type = other DNA
gtttactctcatgtaagtcaacaatgtcctgggattgggacacactttctgggcactgctggccagtcccaaaatggaac

SEQ ID NO: 102 - DNA, 2341 bp, synthetic construct
  misc_feature 1..2341: note = Reporter gene
  source 1..2341: mol_type = other DNA
atagtaatcaattacggggtcattagttcatagcccatatatggagttccgcgttacataacttacggtaaatggcccgcctggctgaccgcccaacgacccccgcccattgacgtcaataatgacgtatgttcccatagtaacgccaatagggactttccattgacgtcaatgggtggagtatttacggtaaactgcccacttggcagtacatcaagtgtatcatatgccaagtccgccccctattgacgtcaatgacggtaaatggcccgcctggcattatgcccagtacatgaccttacgggactttcctacttggcagtacatctacgtattagtcatcgctattaccatggtgatgcggttttggcagtacaccaatgggcgtggatagcggtttgactcacggggatttccaagtctccaccccattgacgtcaatgggagtttgttttggcaccaaaatcaacgggactttccaaaatgtcgtaataaccccgccccgttgacgcaaatgggcggtaggcgtgtacggtgggaggtctatataagcagaggtcgtttagtgaaccgtcagatcacgcgtgctagcactaagacctgaaagggttgtgtctatcagctgcacccctgggtagcgacacaacctcgggaaggcctcagccccctcctcgtacagcactgcctgttggaaagcttgagggaggctatggatgtgcagcacttggcagagggtctggtcatggaagttaccagcaaatatgagctacttttatgattttattttatccaaaagaaagagaatgaaagaagaggggaggaaacaagactaatcaggaaagatgaaggtctaggggtgagggaaggagtaaggagacataaaggcaatgtggagcagctgaggggggaaatggctttcaccacttcccagcatctattgacattgcactctcaaatattttataagactctatattcaaggtaatgtttgaaccctgctgagccagtggcatgggtctctgagagaatcattaacttaatttgactatctggtttgtgggtgcgtttactctcatgtaagtcaacaatgtcctgggattgggacacactttctgggcactgctggccagtcccaaaatggaacataaggaagtggttcttctacttcttttatttctgaaatcaggtaagacatagtttttttaaattataagaattattttttctcccacaatgtagtaaaaatacatatgccatggctttatgtgcaattcatttaatttttgattcatgaaattcccagttcaaaatcttgtatatgattgaaaaattcttaaaaaaataagtttaatttccccgtgaagactgtcacggtgctggaatgaatgggcagaaaaaataatggttgatttttctaatctaaaagagtgtgcctacatgatggccagtctggctgaaaaataaatagccattgtagctaactatgcaaaggatggctaagctcttcgcttggttctcagtttcattaatttatatcatctctgttcaggtgccatgctcccctcactagcaagttgaaacaatgaaataacggatcccccctctccctcccaccgccaccatggtgagcaagggcgaggagctgttcaccggggtggtgcccatcctggtcgagctggacggcgacgtaaacggccacaagttcagcgtgtccggcgagggcgagggcgatgccacctacggcaagctgaccctgaagttcatctgcaccaccggcaagctgcccgtgccctggcccaccctcgtgaccaccctgacctacggcgtgcagtgcttcagccgctaccccgaccacatgaagcagcacgacttcttcaagtccgccatgcccgaaggctacgtccaggagcgcaccatcttcttcaaggacgacggcaactacaagacccgcgccgaggtgaagttcgagggcgacaccctggtgaaccgcatcgagctgaagggcatcgacttcaaggaggacggcaacatcctggggcacaagctggagtacaactacaacagccacaacgtctatatcatggccgacaagcagaagaacggcatcaaggtgaacttcaagatccgccacaacatcgaggacggcagcgtgcagctcgccgaccactaccagcagaacacccccatcggcgacggccccgtgctgctgcccgacaaccactacctgagcacccagtccgccctgagcaaagaccccaacgagaagcgcgatcacatggtcctgctggagttcgtgaccgccgccgggatcactctcggcatggacgagctgtacaagtaa

SEQ ID NO: 103 - DNA, 7110 bp, synthetic construct
  misc_feature 1..7110: note = EpiRegA DNA sequence
  source 1..7110: mol_type = other DNA
atgaaccatgaccaggaatttgaccccccaaaggtttacccacctgtgccagctgagaagaggaagcccatccgcgtgctgtctctctttgatgggattgctacagggctcctggtgctgaaggacctgggcatccaagtggaccgctacattgcctccgaggtgtgtgaggactccatcacggtgggcatggtgcggcaccagggaaagatcatgtacgtcggggacgtccgcagcgtcacacagaagcatatccaggagtggggcccattcgacctggtgattggaggcagtccctgcaatgacctctccattgtcaaccctgcccgcaagggactttatgagggtactggccgcctcttctttgagttctaccgcctcctgcatgatgcgcggcccaaggagggagatgatcgccccttcttctggctctttgagaatgtggtggccatgggcgttagtgacaagagggacatctcgcgatttcttgagtctaaccccgtgatgattgacgccaaagaagtgtctgctgcacacagggcccgttacttctggggtaaccttcctggcatgaacaggcctttggcatccactgtgaatgataagctggagctgcaagagtgtctggagcacggcagaatagccaagttcagcaaagtgaggaccattaccaccaggtcaaactctataaagcagggcaaagaccagcatttccccgtcttcatgaacgagaaggaggacatcctgtggtgcactgaaatggaaagggtgtttggcttccccgtccactacacagacgtctccaacatgagccgcttggcgaggcagagactgctgggccgatcgtggagcgtgccggtcatccgccacctcttcgctccgctgaaggaatattttgcttgtgtgtctagcggcaatagtaacgctaacagccgcgggccgagcttcagcagcggcctggtgccgttaagcttgcgcggcagccatatgggccctatggagatatacaagacagtgtctgcatggaagagacagccagtgcgggtactgagcctcttcagaaacatcgacaaggtactaaagagtttgggcttcttggaaagcggttctggttctgggggaggaacgctgaagtacgtggaagatgtcacaaatgtcgtgaggagagacgtggagaaatggggcccctttgacctggtgtacggctcgacgcagcccctaggcagctcttgtgatcgctgtcccggctggtacatgttccagttccaccggatcctgcagtatgcgctgcctcgccaggagagtcagcggcccttcttctggatattcatggacaatctgctgctgactgaggatgaccaagagacaactacccgcttccttcagacagaggctgtgaccctccaggatgtccgtggcagagactaccagaatgctatgcgggtgtggagcaacattccagggctgaagagcaagcatgcgcccctgaccccaaaggaagaagagtatctgcaagcccaagtcagaagcaggagcaagctggacgccccgaaagttgacctcctggtgaagaactgccttctcccgctgagagagtacttcaagtatttttctcaaaactcacttcctcttggagggccgagctctggcgcacccccaccaagtggagggtctcctgccgggtccccaacatctactgaagaaggcaccagcgaatccgcaacgcccgagtcaggccctggtacctccacagaaccatctgaaggtagtgcgcctggttccccagctggaagccctacttccaccgaagaaggcacgtcaaccgaaccaagtgaaggatctgcccctgggaccagcactgaaccatctgagccaaaaaagaagagaaaggtaatggacaagaagtacagcatcggcctggccatcggcaccaactctgtgggctgggccgtgatcaccgacgagtacaaggtgcccagcaagaaattcaaggtgctgggcaacaccgaccggcacagcatcaagaagaacctgatcggcgccctgctgttcgacagcggagaaacagccgaggccacccggctgaagagaaccgccagaagaagatacaccagacggaagaaccggatctgctatctgcaagagatcttcagcaacgagatggccaaggtggacgacagcttcttccacagactggaagagtccttcctggtggaagaggataagaagcacgagcggcaccccatcttcggcaacatcgtggacgaggtggcctaccacgagaagtaccccaccatctaccacctgagaaagaaactggtggacagcaccgacaaggccgacctgcggctgatctatctggccctggcccacatgatcaagttccggggccacttcctgatcgagggcgacctgaaccccgacaacagcgacgtggacaagctgttcatccagctggtgcagacctacaaccagctgttcgaggaaaaccccatcaacgccagcggcgtggacgccaaggccatcctgtctgccagactgagcaagagcagacggctggaaaatctgatcgcccagctgcccggcgagaagaagaatggcctgttcggcaacctgattgccctgagcctgggcctgacccccaacttcaagagcaacttcgacctggccgaggatgccaaactgcagctgagcaaggacacctacgacgacgacctggacaacctgctggcccagatcggcgaccagtacgccgacctgtttctggccgccaagaacctgtccgacgccatcctgctgagcgacatcctgagagtgaacaccgagatcaccaaggcccccctgagcgcctctatgatcaagagatacgacgagcaccaccaggacctgaccctgctgaaagctctcgtgcggcagcagctgcctgagaagtacaaagagattttcttcgaccagagcaagaacggctacgccggctacatcgatggcggagccagccaggaagagttctacaagttcatcaagcccatcctggaaaagatggacggcaccgaggaactgctcgtgaagctgaacagagaggacctgctgcggaagcagcggaccttcgacaacggcagcatcccccaccagatccacctgggagagctgcacgccattctgcggcggcaggaagatttttacccattcctgaaggacaaccgggaaaagatcgagaagatcctgaccttccgcatcccctactacgtgggccctctggccaggggaaacagcagattcgcctggatgaccagaaagagcgaggaaaccatcaccccctggaacttcgaggaagtggtggacaagggcgccagcgcccagagcttcatcgagcggatgaccaacttcgataagaacctgcccaacgagaaggtgctgcccaagcacagcctgctgtacgagtacttcaccgtgtacaacgagctgaccaaagtgaaatacgtgaccgagggaatgagaaagcccgccttcctgagcggcgagcagaaaaaagccatcgtggacctgctgttcaagaccaaccggaaagtgaccgtgaagcagctgaaagaggactacttcaagaaaatcgagtgcttcgactccgtggaaatctccggcgtggaagatcggttcaacgcctccctgggcacataccacgatctgctgaaaattatcaaggacaaggacttcctggacaatgaggaaaacgaggacattctggaagatatcgtgctgaccctgacactgtttgaggacagagagatgatcgaggaacggctgaaaacctatgcccacctgttcgacgacaaagtgatgaagcagctgaagcggcggagatacaccggctggggcaggctgagccggaagctgatcaacggcatccgggacaagcagtccggcaagacaatcctggatttcctgaagtccgacggcttcgccaacagaaacttcatgcagctgatccacgacgacagcctgacctttaaagaggacatccagaaagcccaggtgtccggccagggcgatagcctgcacgagcacattgccaatctggccggcagccccgccattaagaagggcatcctgcagacagtgaaggtggtggacgagctcgtgaaagtgatgggccggcacaagcccgagaacatcgtgatcgaaatggccagagagaaccagaccacccagaagggacagaagaacagccgcgagagaatgaagcggatcgaagagggcatcaaagagctgggcagccagatcctgaaagaacaccccgtggaaaacacccagctgcagaacgagaagctgtacctgtactacctgcagaatgggcgggatatgtacgtggaccaggaactggacatcaaccggctgtccgactacgatgtggacgctatcgtgcctcagagctttctgaaggacgactccatcgataacaaagtgctgactcggagcgacaagaaccggggcaagagcgacaacgtgccctccgaagaggtcgtgaagaagatgaagaactactggcgccagctgctgaatgccaagctgattacccagaggaagttcgacaatctgaccaaggccgagagaggcggcctgagcgaactggataaggccggcttcatcaagagacagctggtggaaacccggcagatcacaaagcacgtggcacagatcctggactcccggatgaacactaagtacgacgagaacgacaaactgatccgggaagtgaaagtgatcaccctgaagtccaagctggtgtccgatttccggaaggatttccagttttacaaagtgcgcgagatcaacaactaccaccacgcccacgacgcctacctgaacgccgtcgtgggaaccgccctgatcaaaaagtaccctaagctggaaagcgagttcgtgtacggcgactacaaggtgtacgacgtgcggaagatgatcgccaagagcgagcaggaaatcggcaaggctaccgccaagtacttcttctacagcaacatcatgaactttttcaagaccgagattaccctggccaacggcgagatccggaagcggcctctgatcgagacaaacggcgaaacaggcgagatcgtgtgggataagggccgggactttgccaccgtgcggaaagtgctgtctatgccccaagtgaatatcgtgaaaaagaccgaggtgcagacaggcggcttcagcaaagagtctatcctgcccaagaggaacagcgacaagctgatcgccagaaagaaggactgggaccctaagaagtacggcggcttcgacagccccaccgtggcctattctgtgctggtggtggccaaagtggaaaagggcaagtccaagaaactgaagagtgtgaaagagctgctggggatcaccatcatggaaagaagcagcttcgagaagaatcccatcgactttctggaagccaagggctacaaagaagtgaaaaaggacctgatcatcaagctgcctaagtactccctgttcgagctggaaaacggccggaagagaatgctggcctctgccggcgaactgcagaagggaaacgaactggccctgccctccaaatatgtgaacttcctgtacctggccagccactatgagaagctgaagggctcccccgaggataatgagcagaaacagctgtttgtggaacagcacaaacactacctggacgagatcatcgagcagatcagcgagttctccaagagagtgatcctggccgacgctaatctggacaaggtgctgagcgcctacaacaagcacagagacaagcctatcagagagcaggccgagaatatcatccacctgtttaccctgaccaatctgggagcccctgccgccttcaagtactttgacaccaccatcgaccggaagaggtacaccagcaccaaagaggtgctggacgccaccctgatccaccagagcatcaccggcctgtacgagacacggatcgacctgtctcagctgggaggcgacgcctatccctatgacgtgcccgattatgccagcctgggcagcggctcccccaagaaaaaacgcaaggtggaagatcctaagaaaaagcggaaagtggacggcagcggcagcgagacccccggtaccagcgagagcgccacccccgagagccggacactggtgaccttcaaggatgtatttgtggacttcaccagggaggagtggaagctgctggacactgctcagcagatcgtgtacagaaatgtgatgctggagaactataagaacctggtttccttgggttatcagcttactaagccagatgtgatcctccggttggagaagggagaagagcccgtcgacctcgaggctactaacttcagcctgctgaagcaggctggagacgtggaggagaaccctggacctatgcatatgagcgagctgattaaggagaacatgcacatgaagctgtacatggagggcaccgtggacaaccatcacttcaagtgcacatccgagggcgaaggcaagccctacgagggcacccagaccatgagaatcaaggtggtcgagggcggccctctccccttcgccttcgacatcctggctactagcttcctctacggcagcaagaccttcatcaaccacacccagggcatccccgacttcttcaagcagtccttccctgagggcttcacatgggagagagtcaccacatacgaagacgggggcgtgctgaccgctacccaggacaccagcctccaggacggctgcctcatctacaacgtcaagatcagaggggtgaacttcacatccaacggccctgtgatgcagaagaaaacactcggctgggaggccttcaccgagacgctgtaccccgctgacggcggcctggaaggcagaaacgacatggccctgaagctcgtgggcgggagccatctgatcgcaaacatcaagaccacatatagatccaagaaacccgctaagaacctcaagatgcctggcgtctactatgtggactacagactggaaagaatcaaggaggccaacaacgagacctacgtcgagcagcacgaggtggcagtggccagatactgcgacctccctagcaaactggggcacaagcttaattaa

SEQ ID NO: 104 - protein, 2370 aa, synthetic construct
  REGION 1..2370: note = EpiRegA AA sequence
  SITE 2370: note = misc_feature - Xaa =
MNHDQEFDPPKVYPPVPAEKRKPIRVLSLFDGIATGLLVLKDLGIQVDRYIASEVCEDSITVGMVRHQGKIMYVGDVRSVTQKHIQEWGPFDLVIGGSPCNDLSIVNPARKGLYEGTGRLFFEFYRLLHDARPKEGDDRPFFWLFENVVAMGVSDKRDISRFLESNPVMIDAKEVSAAHRARYFWGNLPGMNRPLASTVNDKLELQECLEHGRIAKFSKVRTITTRSNSIKQGKDQHFPVFMNEKEDILWCTEMERVFGFPVHYTDVSNMSRLARQRLLGRSWSVPVIRHLFAPLKEYFACVSSGNSNANSRGPSFSSGLVPLSLRGSHMGPMEIYKTVSAWKRQPVRVLSLFRNIDKVLKSLGFLESGSGSGGGTLKYVEDVTNVVRRDVEKWGPFDLVYGSTQPLGSSCDRCPGWYMFQFHRILQYALPRQESQRPFFWIFMDNLLLTEDDQETTTRFLQTEAVTLQDVRGRDYQNAMRVWSNIPGLKSKHAPLTPKEEEYLQAQVRSRSKLDAPKVDLLVKNCLLPLREYFKYFSQNSLPLGGPSSGAPPPSGGSPAGSPTSTEEGTSESATPESGPGTSTEPSEGSAPGSPAGSPTSTEEGTSTEPSEGSAPGTSTEPSEPKKKRKVMDKKYSIGLAIGTNSVGWAVITDEYKVPSKKFKVLGNTDRHSIKKNLIGALLFDSGETAEATRLKRTARRRYTRRKNRICYLQEIFSNEMAKVDDSFFHRLEESFLVEEDKKHERHPIFGNIVDEVAYHEKYPTIYHLRKKLVDSTDKADLRLIYLALAHMIKFRGHFLIEGDLNPDNSDVDKLFIQLVQTYNQLFEENPINASGVDAKAILSARLSKSRRLENLIAQLPGEKKNGLFGNLIALSLGLTPNFKSNFDLAEDAKLQLSKDTYDDDLDNLLAQIGDQYADLFLAAKNLSDAILLSDILRVNTEITKAPLSASMIKRYDEHHQDLTLLKALVRQQLPEKYKEIFFDQSKNGYAGYIDGGASQEEFYKFIKPILEKMDGTEELLVKLNREDLLRKQRTFDNGSIPHQIHLGELHAILRRQEDFYPFLKDNREKIEKILTFRIPYYVGPLARGNSRFAWMTRKSEETITPWNFEEVVDKGASAQSFIERMTNFDKNLPNEKVLPKHSLLYEYFTVYNELTKVKYVTEGMRKPAFLSGEQKKAIVDLLFKTNRKVTVKQLKEDYFKKIECFDSVEISGVEDRFNASLGTYHDLLKIIKDKDFLDNEENEDILEDIVLTLTLFEDREMIEERLKTYAHLFDDKVMKQLKRRRYTGWGRLSRKLINGIRDKQSGKTILDFLKSDGFANRNFMQLIHDDSLTFKEDIQKAQVSGQGDSLHEHIANLAGSPAIKKGILQTVKVVDELVKVMGRHKPENIVIEMARENQTTQKGQKNSRERMKRIEEGIKELGSQILKEHPVENTQLQNEKLYLYYLQNGRDMYVDQELDINRLSDYDVDAIVPQSFLKDDSIDNKVLTRSDKNRGKSDNVPSEEVVKKMKNYWRQLLNAKLITQRKFDNLTKAERGGLSELDKAGFIKRQLVETRQITKHVAQILDSRMNTKYDENDKLIREVKVITLKSKLVSDFRKDFQFYKVREINNYHHAHDAYLNAVVGTALIKKYPKLESEFVYGDYKVYDVRKMIAKSEQEIGKATAKYFFYSNIMNFFKTEITLANGEIRKRPLIETNGETGEIVWDKGRDFATVRKVLSMPQVNIVKKTEVQTGGFSKESILPKRNSDKLIARKKDWDPKKYGGFDSPTVAYSVLVVAKVEKGKSKKLKSVKELLGITIMERSSFEKNPIDFLEAKGYKEVKKDLIIKLPKYSLFELENGRKRMLASAGELQKGNELALPSKYVNFLYLASHYEKLKGSPEDNEQKQLFVEQHKHYLDEIIEQISEFSKRVILADANLDKVLSAYNKHRDKPIREQAENIIHLFTLTNLGAPAAFKYFDTTIDRKRYTSTKEVLDATLIHQSITGLYETRIDLSQLGGDAYPYDVPDYASLGSGSPKKKRKVEDPKKKRKVDGSGSETPGTSESATPESRTLVTFKDVFVDFTREEWKLLDTAQQIVYRNVMLENYKNLVSLGYQLTKPDVILRLEKGEEPVDLEATNFSLLKQAGDVEENPGPMHMSELIKENMHMKLYMEGTVDNHHFKCTSEGEGKPYEGTQTMRIKVVEGGPLPFAFDILATSFLYGSKTFINHTQGIPDFFKQSFPEGFTWERVTTYEDGGVLTATQDTSLQDGCLIYNVKIRGVNFTSNGPVMQKKTLGWEAFTETLYPADGGLEGRNDMALKLVGGSHLIANIKTTYRSKKPAKNLKMPGVYYVDYRLERIKEANNETYVEQHEVAVARYCDLPSKLGHKLNX

SEQ ID NO: 105 - DNA, 7224 bp, synthetic construct
  misc_feature 1..7224: note = EpiRegB DNA sequence
  source 1..7224: mol_type = other DNA
atgaaccatgaccaggaatttgaccccccaaaggtttacccacctgtgccagctgagaagaggaagcccatccgcgtgctgtctctctttgatgggattgctacagggctcctggtgctgaaggacctgggcatccaagtggaccgctacattgcctccgaggtgtgtgaggactccatcacggtgggcatggtgcggcaccagggaaagatcatgtacgtcggggacgtccgcagcgtcacacagaagcatatccaggagtggggcccattcgacctggtgattggaggcagtccctgcaatgacctctccattgtcaaccctgcccgcaagggactttatgagggtactggccgcctcttctttgagttctaccgcctcctgcatgatgcgcggcccaaggagggagatgatcgccccttcttctggctctttgagaatgtggtggccatgggcgttagtgacaagagggacatctcgcgatttcttgagtctaaccccgtgatgattgacgccaaagaagtgtctgctgcacacagggcccgttacttctggggtaaccttcctggcatgaacaggcctttggcatccactgtgaatgataagctggagctgcaagagtgtctggagcacggcagaatagccaagttcagcaaagtgaggaccattaccaccaggtcaaactctataaagcagggcaaagaccagcatttccccgtcttcatgaacgagaaggaggacatcctgtggtgcactgaaatggaaagggtgtttggcttccccgtccactacacagacgtctccaacatgagccgcttggcgaggcagagactgctgggccgatcgtggagcgtgccggtcatccgccacctcttcgctccgctgaaggaatattttgcttgtgtgtctagcggcaatagtaacgctaacagccgcgggccgagcttcagcagcggcctggtgccgttaagcttgcgcggcagccatatgggccctatggagatatacaagacagtgtctgcatggaagagacagccagtgcgggtactgagcctcttcagaaacatcgacaaggtactaaagagtttgggcttcttggaaagcggttctggttctgggggaggaacgctgaagtacgtggaagatgtcacaaatgtcgtgaggagagacgtggagaaatggggcccctttgacctggtgtacggctcgacgcagcccctaggcagctcttgtgatcgctgtcccggctggtacatgttccagttccaccggatcctgcagtatgcgctgcctcgccaggagagtcagcggcccttcttctggatattcatggacaatctgctgctgactgaggatgaccaagagacaactacccgcttccttcagacagaggctgtgaccctccaggatgtccgtggcagagactaccagaatgctatgcgggtgtggagcaacattccagggctgaagagcaagcatgcgcccctgaccccaaaggaagaagagtatctgcaagcccaagtcagaagcaggagcaagctggacgccccgaaagttgacctcctggtgaagaactgccttctcccgctgagagagtacttcaagtatttttctcaaaactcacttcctcttgacggcagcggcagcgagacccccggtaccagcgagagcgccacccccgagagcatgaacaattcccagggaagagtgaccttcgaggatgtcactgtgaacttcacccagggggagtggcagcggctgaatcccgaacagagaaacttgtacagggatgtgatgctggagaattacagcaaccttgtctctgtgggacaaggggaaaccaccaaacccgatgtgatcttgaggttggaacaaggaaaggagccatggttggaggaagaggaagtgctgggaagtggccgtgcagaaaaaaatggggacattggagggcagatttggaagccaaaggatgtgaaagagagtctcggagggccgagctctggcgcacccccaccaagtggagggtctcctgccgggtccccaacatctactgaagaaggcaccagcgaatccgcaacgcccgagtcaggccctggtacctccacagaaccatctgaaggtagtgcgcctggttccccagctggaagccctacttccaccgaagaaggcacgtcaaccgaaccaagtgaaggatctgcccctgggaccagcactgaaccatctgagccaaaaaagaagagaaaggtaatggacaagaagtacagcatcggcctggccatcggcaccaactctgtgggctgggccgtgatcaccgacgagtacaaggtgcccagcaagaaattcaaggtgctgggcaacaccgaccggcacagcatcaagaagaacctgatcggcgccctgctgttcgacagcggagaaacagccgaggccacccggctgaagagaaccgccagaagaagatacaccagacggaagaaccggatctgctatctgcaagagatcttcagcaacgagatggccaaggtggacgacagcttcttccacagactggaagagtccttcctggtggaagaggataagaagcacgagcggcaccccatcttcggcaacatcgtggacgaggtggcctaccacgagaagtaccccaccatctaccacctgagaaagaaactggtggacagcaccgacaaggccgacctgcggctgatctatctggccctggcccacatgatcaagttccggggccacttcctgatcgagggcgacctgaaccccgacaacagcgacgtggacaagctgttcatccagctggtgcagacctacaaccagctgttcgaggaaaaccccatcaacgccagcggcgtggacgccaaggccatcctgtctgccagactgagcaagagcagacggctggaaaatctgatcgcccagctgcccggcgagaagaagaatggcctgttcggcaacctgattgccctgagcctgggcctgacccccaacttcaagagcaacttcgacctggccgaggatgccaaactgcagctgagcaaggacacctacgacgacgacctggacaacctgctggcccagatcggcgaccagtacgccgacctgtttctggccgccaagaacctgtccgacgccatcctgctgagcgacatcctgagagtgaacaccgagatcaccaaggcccccctgagcgcctctatgatcaagagatacgacgagcaccaccaggacctgaccctgctgaaagctctcgtgcggcagcagctgcctgagaagtacaaagagattttcttcgaccagagcaagaacggctacgccggctacatcgatggcggagccagccaggaagagttctacaagttcatcaagcccatcctggaaaagatggacggcaccgaggaactgctcgtgaagctgaacagagaggacctgctgcggaagcagcggaccttcgacaacggcagcatcccccaccagatccacctgggagagctgcacgccattctgcggcggcaggaagatttttacccattcctgaaggacaaccgggaaaagatcgagaagatcctgaccttccgcatcccctactacgtgggccctctggccaggggaaacagcagattcgcctggatgaccagaaagagcgaggaaaccatcaccccctggaacttcgaggaagtggtggacaagggcgccagcgcccagagcttcatcgagcggatgaccaacttcgataagaacctgcccaacgagaaggtgctgcccaagcacagcctgctgtacgagtacttcaccgtgtacaacgagctgaccaaagtgaaatacgtgaccgagggaatgagaaagcccgccttcctgagcggcgagcagaaaaaagccatcgtggacctgctgttcaagaccaaccggaaagtgaccgtgaagcagctgaaagaggactacttcaagaaaatcgagtgcttcgactccgtggaaatctccggcgtggaagatcggttcaacgcctccctgggcacataccacgatctgctgaaaattatcaaggacaaggacttcctggacaatgaggaaaacgaggacattctggaagatatcgtgctgaccctgacactgtttgaggacagagagatgatcgaggaacggctgaaaacctatgcccacctgttcgacgacaaagtgatgaagcagctgaagcggcggagatacaccggctggggcaggctgagccggaagctgatcaacggcatccgggacaagcagtccggcaagacaatcctggatttcctgaagtccgacggcttcgccaacagaaacttcatgcagctgatccacgacgacagcctgacctttaaagaggacatccagaaagcccaggtgtccggccagggcgatagcctgcacgagcacattgccaatctggccggcagccccgccattaagaagggcatcctgcagacagtgaaggtggtggacgagctcgtgaaagtgatgggccggcacaagcccgagaacatcgtgatcgaaatggccagagagaaccagaccacccagaagggacagaagaacagccgcgagagaatgaagcggatcgaagagggcatcaaagagctgggcagccagatcctgaaagaacaccccgtggaaaacacccagctgcagaacgagaagctgtacctgtactacctgcagaatgggcgggatatgtacgtggaccaggaactggacatcaaccggctgtccgactacgatgtggacgctatcgtgcctcagagctttctgaaggacgactccatcgataacaaagtgctgactcggagcgacaagaaccggggcaagagcgacaacgtgccctccgaagaggtcgtgaagaagatgaagaactactggcgccagctgctgaatgccaagctgattacccagaggaagttcgacaatctgaccaaggccgagagaggcggcctgagcgaactggataaggccggcttcatcaagagacagctggtggaaacccggcagatcacaaagcacgtggcacagatcctggactcccggatgaacactaagtacgacgagaacgacaaactgatccgggaagtgaaagtgatcaccctgaagtccaagctggtgtccgatttccggaaggatttccagttttacaaagtgcgcgagatcaacaactaccaccacgcccacgacgcctacctgaacgccgtcgtgggaaccgccctgatcaaaaagtaccctaagctggaaagcgagttcgtgtacggcgactacaaggtgtacgacgtgcggaagatgatcgccaagagcgagcaggaaatcggcaaggctaccgccaagtacttcttctacagcaacatcatgaactttttcaagaccgagattaccctggccaacggcgagatccggaagcggcctctgatcgagacaaacggcgaaacaggcgagatcgtgtgggataagggccgggactttgccaccgtgcggaaagtgctgtctatgccccaagtgaatatcgtgaaaaagaccgaggtgcagacaggcggcttcagcaaagagtctatcctgcccaagaggaacagcgacaagctgatcgccagaaagaaggactgggaccctaagaagtacggcggcttcgacagccccaccgtggcctattctgtgctggtggtggccaaagtggaaaagggcaagtccaagaaactgaagagtgtgaaagagctgctggggatcaccatcatggaaagaagcagcttcgagaagaatcccatcgactttctggaagccaagggctacaaagaagtgaaaaaggacctgatcatcaagctgcctaagtactccctgttcgagctggaaaacggccggaagagaatgctggcctctgccggcgaactgcagaagggaaacgaactggccctgccctccaaatatgtgaacttcctgtacctggccagccactatgagaagctgaagggctcccccgaggataatgagcagaaacagctgtttgtggaacagcacaaacactacctggacgagatcatcgagcagatcagcgagttctccaagagagtgatcctggccgacgctaatctggacaaggtgctgagcgcctacaacaagcacagagacaagcctatcagagagcaggccgagaatatcatccacctgtttaccctgaccaatctgggagcccctgccgccttcaagtactttgacaccaccatcgaccggaagaggtacaccagcaccaaagaggtgctggacgccaccctgatccaccagagcatcaccggcctgtacgagacacggatcgacctgtctcagctgggaggcgacgcctatccctatgacgtgcccgattatgccagcctgggcagcggctcccccaagaaaaaacgcaaggtggaagatcctaagaaaaagcggaaagtggacggcctcgaggctactaacttcagcctgctgaagcaggctggagacgtggaggagaaccctggacctatgcatgtgagcgagctgattaaggagaacatgcacatgaagctgtacatggagggcaccgtggacaaccatcacttcaagtgcacatccgagggcgaaggcaagccctacgagggcacccagaccatgagaatcaaggtggtcgagggcggccctctccccttcgccttcgacatcctggctactagcttcctctacggcagcaagaccttcatcaaccacacccagggcatccccgacttcttcaagcagtccttccctgagggcttcacatgggagagagtcaccacatacgaagacgggggcgtgctgaccgctacccaggacaccagcctccaggacggctgcctcatctacaacgtcaagatcagaggggtgaacttcacatccaacggccctgtgatgcagaagaaaacactcggctgggaggccttcaccgaaacgctgtaccccgctgacggcggcctggaaggcagaaacgacatggccctgaagctcgtgggcgggagccatctgatcgcaaacatcaagaccacatatagatccaagaaacccgctaagaacctcaagatgcctggcgtctactatgtggactacagactggaaagaatcaaggaggccaacaacgagacctacgtcgagcagcacgaggtggcagtggccagatactgcgacctccctagcaaactggggcacaagcttaattaa

SEQ ID NO: 106 - protein, 2408 aa, synthetic construct
  REGION 1..2408: note = EpiRegB AA sequence
  SITE 2408: note = misc_feature - Xaa =
MNHDQEFDPPKVYPPVPAEKRKPIRVLSLFDGIATGLLVLKDLGIQVDRYIASEVCEDSITVGMVRHQGKIMYVGDVRSVTQKHIQEWGPFDLVIGGSPCNDLSIVNPARKGLYEGTGRLFFEFYRLLHDARPKEGDDRPFFWLFENVVAMGVSDKRDISRFLESNPVMIDAKEVSAAHRARYFWGNLPGMNRPLASTVNDKLELQECLEHGRIAKFSKVRTITTRSNSIKQGKDQHFPVFMNEKEDILWCTEMERVFGFPVHYTDVSNMSRLARQRLLGRSWSVPVIRHLFAPLKEYFACVSSGNSNANSRGPSFSSGLVPLSLRGSHMGPMEIYKTVSAWKRQPVRVLSLFRNIDKVLKSLGFLESGSGSGGGTLKYVEDVTNVVRRDVEKWGPFDLVYGSTQPLGSSCDRCPGWYMFQFHRILQYALPRQESQRPFFWIFMDNLLLTEDDQETTTRFLQTEAVTLQDVRGRDYQNAMRVWSNIPGLKSKHAPLTPKEEEYLQAQVRSRSKLDAPKVDLLVKNCLLPLREYFKYFSQNSLPLDGSGSETPGTSESATPESMNNSQGRVTFEDVTVNFTQGEWQRLNPEQRNLYRDVMLENYSNLVSVGQGETTKPDVILRLEQGKEPWLEEEEVLGSGRAEKNGDIGGQIWKPKDVKESLGGPSSGAPPPSGGSPAGSPTSTEEGTSESATPESGPGTSTEPSEGSAPGSPAGSPTSTEEGTSTEPSEGSAPGTSTEPSEPKKKRKVMDKKYSIGLAIGTNSVGWAVITDEYKVPSKKFKVLGNTDRHSIKKNLIGALLFDSGETAEATRLKRTARRRYTRRKNRICYLQEIFSNEMAKVDDSFFHRLEESFLVEEDKKHERHPIFGNIVDEVAYHEKYPTIYHLRKKLVDSTDKADLRLIYLALAHMIKFRGHFLIEGDLNPDNSDVDKLFIQLVQTYNQLFEENPINASGVDAKAILSARLSKSRRLENLIAQLPGEKKNGLFGNLIALSLGLTPNFKSNFDLAEDAKLQLSKDTYDDDLDNLLAQIGDQYADLFLAAKNLSDAILLSDILRVNTEITKAPLSASMIKRYDEHHQDLTLLKALVRQQLPEKYKEIFFDQSKNGYAGYIDGGASQEEFYKFIKPILEKMDGTEELLVKLNREDLLRKQRTFDNGSIPHQIHLGELHAILRRQEDFYPFLKDNREKIEKILTFRIPYYVGPLARGNSRFAWMTRKSEETITPWNFEEVVDKGASAQSFIERMTNFDKNLPNEKVLPKHSLLYEYFTVYNELTKVKYVTEGMRKPAFLSGEQKKAIVDLLFKTNRKVTVKQLKEDYFKKIECFDSVEISGVEDRFNASLGTYHDLLKIIKDKDFLDNEENEDILEDIVLTLTLFEDREMIEERLKTYAHLFDDKVMKQLKRRRYTGWGRLSRKLINGIRDKQSGKTILDFLKSDGFANRNFMQLIHDDSLTFKEDIQKAQVSGQGDSLHEHIANLAGSPAIKKGILQTVKVVDELVKVMGRHKPENIVIEMARENQTTQKGQKNSRERMKRIEEGIKELGSQILKEHPVENTQLQNEKLYLYYLQNGRDMYVDQELDINRLSDYDVDAIVPQSFLKDDSIDNKVLTRSDKNRGKSDNVPSEEVVKKMKNYWRQLLNAKLITQRKFDNLTKAERGGLSELDKAGFIKRQLVETRQITKHVAQILDSRMNTKYDENDKLIREVKVITLKSKLVSDFRKDFQFYKVREINNYHHAHDAYLNAVVGTALIKKYPKLESEFVYGDYKVYDVRKMIAKSEQEIGKATAKYFFYSNIMNFFKTEITLANGEIRKRPLIETNGETGEIVWDKGRDFATVRKVLSMPQVNIVKKTEVQTGGFSKESILPKRNSDKLIARKKDWDPKKYGGFDSPTVAYSVLVVAKVEKGKSKKLKSVKELLGITIMERSSFEKNPIDFLEAKGYKEVKKDLIIKLPKYSLFELENGRKRMLASAGELQKGNELALPSKYVNFLYLASHYEKLKGSPEDNEQKQLFVEQHKHYLDEIIEQISEFSKRVILADANLDKVLSAYNKHRDKPIREQAENIIHLFTLTNLGAPAAFKYFDTTIDRKRYTSTKEVLDATLIHQSITGLYETRIDLSQLGGDAYPYDVPDYASLGSGSPKKKRKVEDPKKKRKVDGLEATNFSLLKQAGDVEENPGPMHVSELIKENMHMKLYMEGTVDNHHFKCTSEGEGKPYEGTQTMRIKVVEGGPLPFAFDILATSFLYGSKTFINHTQGIPDFFKQSFPEGFTWERVTTYEDGGVLTATQDTSLQDGCLIYNVKIRGVNFTSNGPVMQKKTLGWEAFTETLYPADGGLEGRNDMALKLVGGSHLIANIKTTYRSKKPAKNLKMPGVYYVDYRLERIKEANNETYVEQHEVAVARYCDLPSKLGHKLNX

SEQ ID NO: 107 - DNA, 7446 bp, synthetic construct
  misc_feature 1..7446: note = EpiRegC DNA sequence
  source 1..7446: mol_type = other DNA
atgccaaaaaagaagagaaaggtaatggacaagaagtacagcatcggcctggccatcggcaccaactctgtgggctgggccgtgatcaccgacgagtacaaggtgcccagcaagaaattcaaggtgctgggcaacaccgaccggcacagcatcaagaagaacctgatcggcgccctgctgttcgacagcggagaaacagccgaggccacccggctgaagagaaccgccagaagaagatacaccagacggaagaaccggatctgctatctgcaagagatcttcagcaacgagatggccaaggtggacgacagcttcttccacagactggaagagtccttcctggtggaagaggataagaagcacgagcggcaccccatcttcggcaacatcgtggacgaggtggcctaccacgagaagtaccccaccatctaccacctgagaaagaaactggtggacagcaccgacaaggccgacctgcggctgatctatctggccctggcccacatgatcaagttccggggccacttcctgatcgagggcgacctgaaccccgacaacagcgacgtggacaagctgttcatccagctggtgcagacctacaaccagctgttcgaggaaaaccccatcaacgccagcggcgtggacgccaaggccatcctgtctgccagactgagcaagagcagacggctggaaaatctgatcgcccagctgcccggcgagaagaagaatggcctgttcggcaacctgattgccctgagcctgggcctgacccccaacttcaagagcaacttcgacctggccgaggatgccaaactgcagctgagcaaggacacctacgacgacgacctggacaacctgctggcccagatcggcgaccagtacgccgacctgtttctggccgccaagaacctgtccgacgccatcctgctgagcgacatcctgagagtgaacaccgagatcaccaaggcccccctgagcgcctctatgatcaagagatacgacgagcaccaccaggacctgaccctgctgaaagctctcgtgcggcagcagctgcctgagaagtacaaagagattttcttcgaccagagcaagaacggctacgccggctacatcgatggcggagccagccaggaagagttctacaagttcatcaagcccatcctggaaaagatggacggcaccgaggaactgctcgtgaagctgaacagagaggacctgctgcggaagcagcggaccttcgacaacggcagcatcccccaccagatccacctgggagagctgcacgccattctgcggcggcaggaagatttttacccattcctgaaggacaaccgggaaaagatcgagaagatcctgaccttccgcatcccctactacgtgggccctctggccaggggaaacagcagattcgcctggatgaccagaaagagcgaggaaaccatcaccccctggaacttcgaggaagtggtggacaagggcgccagcgcccagagcttcatcgagcggatgaccaacttcgataagaacctgcccaacgagaaggtgctgcccaagcacagcctgctgtacgagtacttcaccgtgtacaacgagctgaccaaagtgaaatacgtgaccgagggaatgagaaagcccgccttcctgagcggcgagcagaaaaaagccatcgtggacctgctgttcaagaccaaccggaaagtgaccgtgaagcagctgaaagaggactacttcaagaaaatcgagtgcttcgactccgtggaaatctccggcgtggaagatcggttcaacgcctccctgggcacataccacgatctgctgaaaattatcaaggacaaggacttcctggacaatgaggaaaacgaggacattctggaagatatcgtgctgaccctgacactgtttgaggacagagagatgatcgaggaacggctgaaaacctatgcccacctgttcgacgacaaagtgatgaagcagctgaagcggcggagatacaccggctggggcaggctgagccggaagctgatcaacggcatccgggacaagcagtccggcaagacaatcctggatttcctgaagtccgacggcttcgccaacagaaacttcatgcagctgatccacgacgacagcctgacctttaaagaggacatccagaaagcccaggtgtccggccagggcgatagcctgcacgagcacattgccaatctggccggcagccccgccattaagaagggcatcctgcagacagtgaaggtggtggacgagctcgtgaaagtgatgggccggcacaagcccgagaacatcgtgatcgaaatggccagagagaaccagaccacccagaagggacagaagaacagccgcgagagaatgaagcggatcgaagagggcatcaaagagctgggcagccagatcctgaaagaacaccccgtggaaaacacccagctgcagaacgagaagctgtacctgtactacctgcagaatgggcgggatatgtacgtggaccaggaactggacatcaaccggctgtccgactacgatgtggacgctatcgtgcctcagagctttctgaaggacgactccatcgataacaaagtgctgactcggagcgacaagaaccggggcaagagcgacaacgtgccctccgaagaggtcgtgaagaagatgaagaactactggcgccagctgctgaatgccaagctgattacccagaggaagttcgacaatctgaccaaggccgagagaggcggcctgagcgaactggataaggccggcttcatcaagagacagctggtggaaacccggcagatcacaaagcacgtggcacagatcctggactcccggatgaacactaagtacgacgagaacgacaaactgatccgggaagtgaaagtgatcaccctgaagtccaagctggtgtccgatttccggaaggatttccagttttacaaagtgcgcgagatcaacaactaccaccacgcccacgacgcctacctgaacgccgtcgtgggaaccgccctgatcaaaaagtaccctaagctggaaagcgagttcgtgtacggcgactacaaggtgtacgacgtgcggaagatgatcgccaagagcgagcaggaaatcggcaaggctaccgccaagtacttcttctacagcaacatcatgaactttttcaagaccgagattaccctggccaacggcgagatccggaagcggcctctgatcgagacaaacggcgaaacaggcgagatcgtgtgggataagggccgggactttgccaccgtgcggaaagtgctgtctatgccccaagtgaatatcgtgaaaaagaccgaggtgcagacaggcggcttcagcaaagagtctatcctgcccaagaggaacagcgacaagctgatcgccagaaagaaggactgggaccctaagaagtacggcggcttcgacagccccaccgtggcctattctgtgctggtggtggccaaagtggaaaagggcaagtccaagaaactgaagagtgtgaaagagctgctggggatcaccatcatggaaagaagcagcttcgagaagaatcccatcgactttctggaagccaagggctacaaagaagtgaaaaaggacctgatcatcaagctgcctaagtactccctgttcgagctggaaaacggccggaagagaatgctggcctctgccggcgaactgcagaagggaaacgaactggccctgccctccaaatatgtgaacttcctgtacctggccagccactatgagaagctgaagggctcccccgaggataatgagcagaaacagctgtttgtggaacagcacaaacactacctggacgagatcatcgagcagatcagcgagttctccaagagagtgatcctggccgacgctaatctggacaaggtgctgagcgcctacaacaagcacagagacaagcctatcagagagcaggccgagaatatcatccacctgtttaccctgaccaatctgggagcccctgccgccttcaagtactttgacaccaccatcgaccggaagaggtacaccagcaccaaagaggtgctggacgccaccctgatccaccagagcatcaccggcctgtacgagacacggatcgacctgtctcagctgggaggcgacgcctatccctatgacgtgcccgattatgccagcctgggcagcggctcccccaagaaaaaacgcaaggtggaagatcctaagaaaaagcggaaagtggacggcggagggccgagctctggcgcacccccaccaagtggagggtctcctgccgggtccccaacatctactgaagaaggcaccagcgaatccgcaacgcccgagtcaggccctggtacctccacagaaccatctgaaggtagtgcgcctggttccccagctggaagccctacttccaccgaagaaggcacgtcaaccgaaccaagtgaaggatctgcccctgggaccagcactgaaccatctgagatgaacaattcccagggaagagtgaccttcgaggacgtgaccgtgaacttcacccaaggcgagtggcagagactgaaccccgagcagagaaacctgtaccgggacgtgatgctggaaaactacagcaacctggtgtccgtcggccagggcgagacaacaaagcctgacgtgatcctgcggctggaacagggcaaagagccttggctggaagaggaagaggtgctcggatctggcagagccgagaagaatggcgatatcggcggacagatctggaagccaaaggatgtgaaagagagtctcagcggcagcgagacccccggtaccagcgagggcggccctagcagcggcgcccctccccctagcggcggcagccctgccggatcccctacaagcaccgaagaaggcacaagcgagtccgctacccctgagtccggccctggcacctccacagagcctagcgagggatccgctcctggatcccctgccggaagccctacctccaccgaggagggcacaagcaccgagccttccgagggcagcgcccccggaacaagcaccgaacctagcgagagcgccacccccgagagcatgttcgaaaccgtgcctgtgtggaggagacagccagtccgggtgctgtccctttttgaagacatcaagaaagagctgacgagtttgggctttttggaaagtggttctgacccgggacaactgaagcatgtggttgatgtcacagacacagtgaggaaggatgtggaggagtggggacccttcgatcttgtgtacggcgccacacctcccctgggccacacctgtgaccgtcctcccagctggtacctgttccagttccaccggctcctgcagtacgcacggcccaagccaggcagccccaggcccttcttctggatgttcgtggacaatctggtgctgaacaaggaagacctggacgtcgcatctcgcttcctggagatggagccagtcaccatcccagatgtccacggcggatccttgcagaatgctgtccgcgtgtggagcaacatcccagccataaggagcagcaggcactgggctctggtttcggaagaagaattgtccctgctggcccagaacaagcagagctcgaagctcgcggccaagtggcccaccaagctggtgaagaactgctttctccccctaagagaatatttcaagtatttttcaacagaactcacttcctctttatctagcggcaatagtaacgctaacagccgcgggccgagcttcagcagcggcctggtgccgttaagcttgcgcggcagccatatgaaccatgaccaggaatttgaccccccaaaggtttacccacctgtgccagctgagaagaggaagcccatccgcgtgctgtctctctttgatgggattgctacagggctcctggtgctgaaggacctgggcatccaagtggaccgctacattgcctccgaggtgtgtgaggactccatcacggtgggcatggtgcggcaccagggaaagatcatgtacgtcggggacgtccgcagcgtcacacagaagcatatccaggagtggggcccattcgacctggtgattggaggcagtccctgcaatgacctctccattgtcaaccctgcccgcaagggactttatgagggtactggccgcctcttctttgagttctaccgcctcctgcatgatgcgcggcccaaggagggagatgatcgccccttcttctggctctttgagaatgtggtggccatgggcgttagtgacaagagggacatctcgcgatttcttgagtctaaccccgtgatgattgacgccaaagaagtgtctgctgcacacagggcccgttacttctggggtaaccttcctggcatgaacaggcctttggcatccactgtgaatgataagctggagctgcaagagtgtctggagcacggcagaatagccaagttcagcaaagtgaggaccattaccaccaggtcaaactctataaagcagggcaaagaccagcatttccccgtcttcatgaacgagaaggaggacatcctgtggtgcactgaaatggaaagggtgtttggcttccccgtccactacacagacgtctccaacatgagccgcttggcgaggcagagactgctgggccgatcgtggagcgtgccggtcatccgccacctcttcgctccgctgaaggaatattttgcttgtgtgctcgaggctactaacttcagcctgctgaagcaggctggagacgtggaggagaaccctggacctatgcatgtgagcgagctgattaaggagaacatgcacatgaagctgtacatggagggcaccgtggacaaccatcacttcaagtgcacatccgagggcgaaggcaagccctacgagggcacccagaccatgagaatcaaggtggtcgagggcggccctctccccttcgccttcgacatcctggctactagcttcctctacggcagcaagaccttcatcaaccacacccagggcatccccgacttcttcaagcagtccttccctgagggcttcacatgggagagagtcaccacatacgaagacgggggcgtgctgaccgctacccaggacaccagcctccaggacggctgcctcatctacaacgtcaagatcagaggggtgaacttcacatccaacggccctgtgatgcagaagaaaacactcggctgggaggccttcaccgaaacgctgtaccccgctgacggcggcctggaaggcagaaacgacatggccctgaagctcgtgggcgggagccatctgatcgcaaacatcaagaccacatatagatccaagaaacccgctaagaacctcaagatgcctggcgtctactatgtggactacagactggaaagaatcaaggaggccaacaacgagacctacgtcgagcagcacgaggtggcagtggccagatactgcgacctccctagcaaactggggcacaagcttaattaa

SEQ ID NO: 108 - protein, 2482 aa, synthetic construct
  REGION 1..2482: note = EpiRegC AA sequence
  SITE 2482: note = misc_feature - Xaa =
MPKKKRKVMDKKYSIGLAIGTNSVGWAVITDEYKVPSKKFKVLGNTDRHSIKKNLIGALLFDSGETAEATRLKRTARRRYTRRKNRICYLQEIFSNEMAKVDDSFFHRLEESFLVEEDKKHERHPIFGNIVDEVAYHEKYPTIYHLRKKLVDSTDKADLRLIYLALAHMIKFRGHFLIEGDLNPDNSDVDKLFIQLVQTYNQLFEENPINASGVDAKAILSARLSKSRRLENLIAQLPGEKKNGLFGNLIALSLGLTPNFKSNFDLAEDAKLQLSKDTYDDDLDNLLAQIGDQYADLFLAAKNLSDAILLSDILRVNTEITKAPLSASMIKRYDEHHQDLTLLKALVRQQLPEKYKEIFFDQSKNGYAGYIDGGASQEEFYKFIKPILEKMDGTEELLVKLNREDLLRKQRTFDNGSIPHQIHLGELHAILRRQEDFYPFLKDNREKIEKILTFRIPYYVGPLARGNSRFAWMTRKSEETITPWNFEEVVDKGASAQSFIERMTNFDKNLPNEKVLPKHSLLYEYFTVYNELTKVKYVTEGMRKPAFLSGEQKKAIVDLLFKTNRKVTVKQLKEDYFKKIECFDSVEISGVEDRFNASLGTYHDLLKIIKDKDFLDNEENEDILEDIVLTLTLFEDREMIEERLKTYAHLFDDKVMKQLKRRRYTGWGRLSRKLINGIRDKQSGKTILDFLKSDGFANRNFMQLIHDDSLTFKEDIQKAQVSGQGDSLHEHIANLAGSPAIKKGILQTVKVVDELVKVMGRHKPENIVIEMARENQTTQKGQKNSRERMKRIEEGIKELGSQILKEHPVENTQLQNEKLYLYYLQNGRDMYVDQELDINRLSDYDVDAIVPQSFLKDDSIDNKVLTRSDKNRGKSDNVPSEEVVKKMKNYWRQLLNAKLITQRKFDNLTKAERGGLSELDKAGFIKRQLVETRQITKHVAQILDSRMNTKYDENDKLIREVKVITLKSKLVSDFRKDFQFYKVREINNYHHAHDAYLNAVVGTALIKKYPKLESEFVYGDYKVYDVRKMIAKSEQEIGKATAKYFFYSNIMNFFKTEITLANGEIRKRPLIETNGETGEIVWDKGRDFATVRKVLSMPQVNIVKKTEVQTGGFSKESILPKRNSDKLIARKKDWDPKKYGGFDSPTVAYSVLVVAKVEKGKSKKLKSVKELLGITIMERSSFEKNPIDFLEAKGYKEVKKDLIIKLPKYSLFELENGRKRMLASAGELQKGNELALPSKYVNFLYLASHYEKLKGSPEDNEQKQLFVEQHKHYLDEIIEQISEFSKRVILADANLDKVLSAYNKHRDKPIREQAENIIHLFTLTNLGAPAAFKYFDTTIDRKRYTSTKEVLDATLIHQSITGLYETRIDLSQLGGDAYPYDVPDYASLGSGSPKKKRKVEDPKKKRKVDGGGPSSGAPPPSGGSPAGSPTSTEEGTSESATPESGPGTSTEPSEGSAPGSPAGSPTSTEEGTSTEPSEGSAPGTSTEPSEMNNSQGRVTFEDVTVNFTQGEWQRLNPEQRNLYRDVMLENYSNLVSVGQGETTKPDVILRLEQGKEPWLEEEEVLGSGRAEKNGDIGGQIWKPKDVKESLSGSETPGTSEGGPSSGAPPPSGGSPAGSPTSTEEGTSESATPESGPGTSTEPSEGSAPGSPAGSPTSTEEGTSTEPSEGSAPGTSTEPSESATPESMFETVPVWRRQPVRVLSLFEDIKKELTSLGFLESGSDPGQLKHVVDVTDTVRKDVEEWGPFDLVYGATPPLGHTCDRPPSWYLFQFHRLLQYARPKPGSPRPFFWMFVDNLVLNKEDLDVASRFLEMEPVTIPDVHGGSLQNAVRVWSNIPAIRSSRHWALVSEEELSLLAQNKQSSKLAAKWPTKLVKNCFLPLREYFKYFSTELTSSLSSGNSNANSRGPSFSSGLVPLSLRGSHMNHDQEFDPPKVYPPVPAEKRKPIRVLSLFDGIATGLLVLKDLGIQVDRYIASEVCEDSITVGMVRHQGKIMYVGDVRSVTQKHIQEWGPFDLVIGGSPCNDLSIVNPARKGLYEGTGRLFFEFYRLLHDARPKEGDDRPFFWLFENVVAMGVSDKRDISRFLESNPVMIDAKEVSAAHRARYFWGNLPGMNRPLASTVNDKLELQECLEHGRIAKFSKVRTITTRSNSIKQGKDQHFPVFMNEKEDILWCTEMERVFGFPVHYTDVSNMSRLARQRLLGRSWSVPVIRHLFAPLKEYFACVLEATNFSLLKQAGDVEENPGPMHVSELIKENMHMKLYMEGTVDNHHFKCTSEGEGKPYEGTQTMRIKVVEGGPLPFAFDILATSFLYGSKTFINHTQGIPDFFKQSFPEGFTWERVTTYEDGGVLTATQDTSLQDGCLIYNVKIRGVNFTSNGPVMQKKTLGWEAFTETLYPADGGLEGRNDMALKLVGGSHLIANIKTTYRSKKPAKNLKMPGVYYVDYRLERIKEANNETYVEQHEVAVARYCDLPSKLGHKLNX

SEQ ID NO: 109 - DNA, 7539 bp, synthetic construct
  misc_feature 1..7539: note = EpiRegA-C vector
  source 1..7539: mol_type = other DNA
gtcgacaatcaacctctggattacaaaatttgtgaaagattgactggtattcttaactatgttgctccttttacgctatgtggatacgctgctttaatgcctttgtatcatgctattgcttcccgtatggctttcattttctcctccttgtataaatcctggttgctgtctctttatgaggagttgtggcccgttgtcaggcaacgtggcgtggtgtgcactgtgtttgctgacgcaacccccactggttggggcattgccaccacctgtcagctcctttccgggactttcgctttccccctccctattgccacggcggaactcatcgccgcctgccttgcccgctgctggacaggggctcggctgttgggcactgacaattccgtggtgttgtcggggaaatcatcgtcctttccttggctgctcgcctgtgttgccacctggattctgcgcgggacgtccttctgctacgtcccttcggccctcaatccagcggaccttccttcccgcggcctgctgccggctctgcggcctcttccgcgtcttcgccttcgccctcagacgagtcggatctccctttgggccgcctccccgcctggtacctttaagaccaatgacttacaaggcagctgtagatcttagccactttttaaaagaaaaggggggactggaagggctaattcactcccaacgaaaataagatctgctttttgcttgtactgggtctctctggttagaccagatctgagcctgggagctctctggctaactagggaacccactgcttaagcctcaataaagcttgccttgagtgcttcaagtagtgtgtgcccgtctgttgtgtgactctggtaactagagatccctcagacccttttagtcagtgtggaaaatctctagcagtagtagttcatgtcatcttattattcagtatttataacttgcaaagaaatgaatatcagagagtgagaggaacttgtttattgcagcttataatggttacaaataaagcaatagcatcacaaatttcacaaataaagcatttttttcactgcattctagttgtggtttgtccaaactcatcaatgtatcttatcatgtctggctctagctatcccgcccctaactccgcccagttccgcccattctccgccccatggctgactaattttttttatttatgcagaggccgaggccgcctcggcctctgagctattccagaagtagtgaggaggcttttttggaggcctagacttttgcagagacggcccaaattcgtaatcatggtcatagctgtttcctgtgtgaaattgttatccgctcacaattccacacaacatacgagccggaagcataaagtgtaaagcctggggtgcctaatgagtgagctaactcacattaattgcgttgcgctcactgcccgctttccagtcgggaaacctgtcgtgccagctgcattaatgaatcggccaacgcgcggggagaggcggtttgcgtattgggcgctcttccgcttcctcgctcactgactcgctgcgctcggtcgttcggctgcggcgagcggtatcagctcactcaaaggcggtaatacggttatccacagaatcaggggataacgcaggaaagaacatgtgagcaaaaggccagcaaaaggccaggaaccgtaaaaaggccgcgttgctggcgtttttccataggctccgcccccctgacgagcatcacaaaaatcgacgctcaagtcagaggtggcgaaacccgacaggactataaagataccaggcgtttccccctggaagctccctcgtgcgctctcctgttccgaccctgccgcttaccggatacctgtccgcctttctcccttcgggaagcgtggcgctttctcatagctcacgctgtaggtatctcagttcggtgtaggtcgttcgctccaagctgggctgtgtgcacgaaccccccgttcagcccgaccgctgcgccttatccggtaactatcgtcttgagtccaacccggtaagacacgacttatcgccactggcagcagccactggtaacaggattagcagagcgaggtatgtaggcggtgctacagagttcttgaagtggtggcctaactacggctacactagaaggacagtatttggtatctgcgctctgctgaagccagttaccttcggaaaaagagttggtagctcttgatccggcaaacaaaccaccgctggtagcggtggtttttttgtttgcaagcagcagattacgcgcagaaaaaaaggatctcaagaagatcctttgatcttttctacggggtctgacgctcagtggaacgaaaactcacgttaagggattttggtcatgagattatcaaaaaggatcttcacctagatccttttaaattaaaaatgaagttttaaatcaatctaaagtatatatgagtaaacttggtctgacagttaccaatgcttaatcagtgaggcacctatctcagcgatctgtctatttcgttcatccatagttgcctgactccccgtcgtgtagataactacgatacgggagggcttaccatctggccccagtgctgcaatgataccgcgagacccacgctcaccggctccagatttatcagcaataaaccagccagccggaagggccgagcgcagaagtggtcctgcaactttatccgcctccatccagtctattaattgttgccgggaagctagagtaagtagttcgccagttaatagtttgcgcaacgttgttgccattgctacaggcatcgtggtgtcacgctcgtcgtttggtatggcttcattcagctccggttcccaacgatcaaggcgagttacatgatcccccatgttgtgcaaaaaagcggttagctccttcggtcctccgatcgttgtcagaagtaagttggccgcagtgttatcactcatggttatggcagcactgcataattctcttactgtcatgccatccgtaagatgcttttctgtgactggtgagtactcaaccaagtcattctgagaatagtgtatgcggcgaccgagttgctcttgcccggcgtcaatacgggataataccgcgccacatagcagaactttaaaagtgctcatcattggaaaacgttcttcggggcgaaaactctcaaggatcttaccgctgttgagatccagttcgatgtaacccactcgtgcacccaactgatcttcagcatcttttactttcaccagcgtttctgggtgagcaaaaacaggaaggcaaaatgccgcaaaaaagggaataagggcgacacggaaatgttgaatactcatactcttcctttttcaatattattgaagcatttatcagggttattgtctcatgagcggatacatatttgaatgtatttagaaaaataaacaaataggggttccgcgcacatttccccgaaaagtgccacctgacgtctaagaaaccattattatcatgacattaacctataaaaataggcgtatcacgaggccctttcgtctcgcgcgtttcggtgatgacggtgaaaacctctgacacatgcagctcccggagacggtcacagcttgtctgtaagcggatgccgggagcagacaagcccgtcagggcgcgtcagcgggtgttggcgggtgtcggggctggcttaactatgcggcatcagagcagattgtactgagagtgcaccatatgcggtgtgaaataccgcacagatgcgtaaggagaaaataccgcatcaggcgccattcgccattcaggctgcgcaactgttgggaagggcgatcggtgcgggcctcttcgctattacgccagctggcgaaagggggatgtgctgcaaggcgattaagttgggtaacgccagggttttcccagtcacgacgttgtaaaacgacggccagtgccaagctgacgcgtgtagtcttatgcaatactcttgtagtcttgcaacatggtaacgatgagttagcaacatgccttacaaggagagaaaaagcaccgtgcatgccgattggtggaagtaaggtggtacgatcgtgccttattaggaaggcaacagacgggtctgacatggattggacgaaccactgaattgccgcattgcagagatattgtatttaagtgcctagctcgatacaataaacgggtctctctggttagaccagatctgagcctgggagctctctggctaactagggaacccactgcttaagcctcaataaagcttgccttgagtgcttcaagtagtgtgtgcccgtctgttgtgtgactctggtaactagagatccctcagacccttttagtcagtgtggaaaatctctagcagtggcgcccgaacagggacctgaaagcgaaagggaaaccagagctctctcgacgcaggactcggcttgctgaagcgcgcacggcaagaggcgaggggcggcgactggtgagtacgccaaaaattttgactagcggaggctagaaggagagagatgggtgcgagagcgtcagtattaagcgggggagaattagatcgcgatgggaaaaaattcggttaaggccagggggaaagaaaaaatataaattaaaacatatagtatgggcaagcagggagctagaacgattcgcagttaatcctggcctgttagaaacatcagaaggctgtagacaaatactgggacagctacaaccatcccttcagacaggatcagaagaacttagatcattatataatacagtagcaaccctctattgtgtgcatcaaaggatagagataaaagacaccaaggaagctttagacaagatagaggaagagcaaaacaaaagtaagaccaccgcacagcaagcggccactgatcttcagacctggaggaggagatatgagggacaattggagaagtgaattatataaatataaagtagtaaaaattgaaccattaggagtagcacccaccaaggcaaagagaagagtggtgcagagagaaaaaagagcagtgggaataggagctttgttccttgggttcttgggagcagcaggaagcactatgggcgcagcctcaatgacgctgacggtacaggccagacaattattgtctggtatagtgcagcagcagaacaatttgctgagggctattgaggcgcaacagcatctgttgcaactcacagtctggggcatcaagcagctccaggcaagaatcctggctgtggaaagatacctaaaggatcaacagctcctggggatttggggttgctctggaaaactcatttgcaccactgctgtgccttggaatgctagttggagtaataaatctctggaacagattggaatcacacgacctggatggagtgggacagagaaattaacaattacacaagcttaatacactccttaattgaagaatcgcaaaaccagcaagaaaagaatgaacaagaattattggaattagataaatgggcaagtttgtggaattggtttaacataacaaattggctgtggtatataaaattattcataatgatagtaggaggcttggtaggtttaagaatagtttttgctgtactttctatagtgaatagagttaggcagggatattcaccattatcgtttcagacccacctcccaaccccgaggggacccgacaggcccgaaggaatagaagaagaaggtggagagagagacagagacagatccattcgattagtgaacggatctcgacggttaacttttaaaagaaaaggggggattggggggtacagtgcaggggaaagaatagtagacataatagcaacagacatacaaactaaagaattacaaaaacaaattacaaaaattcaaaattttatcgatactagtggcgcgccggattcgacattgattattgactagttattaatagtaatcaattacggggtcattagttcatagcccatatatggagttccgcgttacataacttacggtaaatggcccgcctggctgaccgcccaacgacccccgcccattgacgtcaataatgacgtatgttcccatagtaacgccaatagggactttccattgacgtcaatgggtggagtatttacggtaaactgcccacttggcagtacatcaagtgtatcatatgccaagtacgccccctattgacgtcaatgacggtaaatggcccgcctggcattatgcccagtacatgaccttatgggactttcctacttggcagtacatctacgtattagtcatcgctattaccatggtcgaggtgagccccacgttctgcttcactctccccatctcccccccctccccacccccaattttgtatttatttattttttaattattttgtgcagcgatgggggcggggggggggggggggcgcgcgccaggcggggcggggcggggcgaggggcggggcggggcgaggcggagaggtgcggcggcagccaatcagagcggcgcgctccgaaagtttccttttatggcgaggcggcggcggcggcggccctataaaaagcgaagcgcgcggcgggcgggagtcgctgcgttgccttcgccccgtgccccgctccgcgccgcctcgcgccgcccgccccggctctgactgaccgcgttactcccacaggtgagcgggcgggacggcccttctcctccgggctgtaattagcgcttggtttaatgacggctcgtttcttttctgtggctgcgtgaaagccttaaagggctccgggagggccctttgtgcgggggggagcggctcggggggtgcgtgcgtgtgtgtgtgcgtggggagcgccgcgtgcggcccgcgctgcccggcggctgtgagcgctgcgggcgcggcgcggggctttgtgcgctccgcgtgtgcgcgaggggagcgcggccgggggcggtgccccgcggtgcgggggggctgcgaggggaacaaaggctgcgtgcggggtgtgtgcgtgggggggtgagcagggggtgtgggcgcggcggtcgggctgtaacccccccctgcacccccctccccgagttgctgagcacggcccggcttcgggtgcggggctccgtgcggggcgtggcgcggggctcgccgtgccgggcggggggtggcggcaggtgggggtgccgggcggggcggggccgcctcgggccggggagggctcgggggaggggcgcggcggccccggagcgccggcggctgtcgaggcgcggcgagccgcagccattgccttttatggtaatcgtgcgagagggcgcagggacttcctttgtcccaaatctggcggagccgaaatctgggaggcgccgccgcaccccctctagcgggcgcgggcgaagcggtgcggcgccggcaggaaggaaatgggcggggagggccttcgtgcgtcgccgcgccgccgtccccttctccatctccagcctcggggctgccgcagggggacggctgccttcgggggggacggggcagggcggggttcggcttctggcgtgtgaccggcggctctagagcctctgctaaccatgttcatgccttcttctttttcctacagatccttaattaagccacc

SEQ ID NO: 110 - DNA, 9144 bp, synthetic construct
  misc_feature 1..9144: note = gRNA vector
  source 1..9144: mol_type = other DNA
gttttagagctagaaatagcaagttaaaataaggctagtccgttatcaacttgaaaaagtggcaccgagtcggtgcttttttgaattcgctagcgagttccgcgttacataacttacggtaaatggcccgcctggctgaccgcccaacgacccccgcccattgacgtcaataatgacgtatgttcccatagtaacgccaatagggactttccattgacgtcaatgggtggagtatttacggtaaactgcccacttggcagtacatcaagtgtatcatatgccaagtccgccccctattgacgtcaatgacggtaaatggcccgcctggcattatgcccagtacatgaccttacgggactttcctacttggcagtacatctacgtattagtcatcgctattaccatggtgatgcggttttggcagtacaccaatgggcgtggatagcggtttgactcacggggatttccaagtctccaccccattgacgtcaatgggagtttgttttggcaccaaaatcaacgggactttccaaaatgtcgtaataaccccgccccgttgacgcaaatgggcggtaggcgtgtacggtgggaggtctatataagcagaggtcgtttagtgaaccgtcagatcacgcgtgccaccatggtgagcaagggcgaggaggataacatggccatcatcaaggagttcatgcgcttcaaggtgcacatggagggctccgtgaacggccacgagttcgagatcgagggcgagggcgagggccgcccctacgagggcacccagaccgccaagctgaaggtgaccaagggtggccccctgcccttcgcctgggacatcctgtcccctcagttcatgtacggctccaaggcctacgtgaagcaccccgccgacatccccgactacttgaagctgtccttccccgagggcttcaagtgggagcgcgtgatgaacttcgaggacggcggcgtggtgaccgtgacccaggactcctccctgcaggacggcgagttcatctacaaggtgaagctgcgcggcaccaacttcccctccgacggccccgtaatgcagaagaagaccatgggctgggaggcctcctccgagcggatgtaccccgaggacggcgccctgaagggcgagatcaagcagaggctgaagctgaaggacggcggccactacgacgctgaggtcaagaccacctacaaggccaagaagcccgtgcagctgcccggcgcctacaacgtcaacatcaagttggacatcacctcccacaacgaggactacaccatcgtggaacagtacgaacgcgccgagggccgccactccaccggcggcatggacgagctgtacaagtaagaattcgatatcaagcttatcgataatcaacctctggattacaaaatttgtgaaagattgactggtattcttaactatgttgctccttttacgctatgtggatacgctgctttaatgcctttgtatcatgctattgcttcccgtatggctttcattttctcctccttgtataaatcctggttgctgtctctttatgaggagttgtggcccgttgtcaggcaacgtggcgtggtgtgcactgtgtttgctgacgcaacccccactggttggggcattgccaccacctgtcagctcctttccgggactttcgctttccccctccctattgccacggcggaactcatcgccgcctgccttgcccgctgctggacaggggctcggctgttgggcactgacaattccgtggtgttgtcggggaaatcatcgtcctttccttggctgctcgcctgtgttgccacctggattctgcgcgggacgtccttctgctacgtcccttcggccctcaatccagcggaccttccttcccgcggcctgctgccggctctgcggcctcttccgcgtcttcgccttcgccctcagacgagtcggatctccctttgggccgcctccccgcgtcgactttaagaccaatgacttacaaggcagctgtagatcttagccactttttaaaagaaaaggggggactggaagggctaattcactcccaacgaagacaagatctgctttttgcttgtactgggtctctctggttagaccagatctgagcctgggagctctctggctaactagggaacccactgcttaagcctcaataaagcttgccttgagtgcttcaagtagtgtgtgcccgtctgttgtgtgactctggtaactagagatccctcagacccttttagtcagtgtggaaaatctctagcagggcccgtttaaacccgctgatcagcctcgactgtgccttctagttgccagccatctgttgtttgcccctcccccgtgccttccttgaccctggaaggtgccactcccactgtcctttcctaataaaatgaggaaattgcatcgcattgtctgagtaggtgtcattctattctggggggtggggtggggcaggacagcaagggggaggattgggaagacaatagcaggcatgctggggatgcggtgggctctatggcttctgaggcggaaagaaccagctggggctctagggggtatccccacgcgccctgtagcggcgcattaagcgcggcgggtgtggtggttacgcgcagcgtgaccgctacacttgccagcgccctagcgcccgctcctttcgctttcttcccttcctttctcgccacgttcgccggctttccccgtcaagctctaaatcgggggctccctttagggttccgatttagtgctttacggcacctcgaccccaaaaaacttgattagggtgatggttcacgtagtgggccatcgccctgatagacggtttttcgccctttgacgttggagtccacgttctttaatagtggactcttgttccaaactggaacaacactcaaccctatctcggtctattcttttgatttataagggattttgccgatttcggcctattggttaaaaaatgagctgatttaacaaaaatttaacgcgaattaattctgtggaatgtgtgtcagttagggtgtggaaagtccccaggctccccagcaggcagaagtatgcaaagcatgcatctcaattagtcagcaaccaggtgtggaaagtccccaggctccccagcaggcagaagtatgcaaagcatgcatctcaattagtcagcaaccatagtcccgcccctaactccgcccatcccgcccctaactccgcccagttccgcccattctccgccccatggctgactaattttttttatttatgcagaggccgaggccgcctctgcctctgagctattccagaagtagtgaggaggcttttttggaggcctaggcttttgcaaaaagctcccgggagcttgtatatccattttcggatctgatcagcacgtgttgacaattaatcatcggcatagtatatcggcatagtataatacgacaaggtgaggaactaaaccatggccaagttgaccagtgccgttccggtgctcaccgcgcgcgacgtcgccggagcggtcgagttctggaccgaccggctcgggttctcccgggacttcgtggaggacgacttcgccggtgtggtccgggacgacgtgaccctgttcatcagcgcggtccaggaccaggtggtgccggacaacaccctggcctgggtgtgggtgcgcggcctggacgagctgtacgccgagtggtcggaggtcgtgtccacgaacttccgggacgcctccgggccggccatgaccgagatcggcgagcagccgtgggggcgggagttcgccctgcgcgacccggccggcaactgcgtgcacttcgtggccgaggagcaggactgacacgtgctacgagatttcgattccaccgccgccttctatgaaaggttgggcttcggaatcgttttccgggacgccggctggatgatcctccagcgcggggatctcatgctggagttcttcgcccaccccaacttgtttattgcagcttataatggttacaaataaagcaatagcatcacaaatttcacaaataaagcatttttttcactgcattctagttgtggtttgtccaaactcatcaatgtatcttatcatgtctgtataccgtcgacctctagctagagcttggcgtaatcatggtcatagctgtttcctgtgtgaaattgttatccgctcacaattccacacaacatacgagccggaagcataaagtgtaaagcctggggtgcctaatgagtgagctaactcacattaattgcgttgcgctcactgcccgctttccagtcgggaaacctgtcgtgccagctgcattaatgaatcggccaacgcgcggggagaggcggtttgcgtattgggcgctcttccgcttcctcgctcactgactcgctgcgctcggtcgttcggctgcggcgagcggtatcagctcactcaaaggcggtaatacggttatccacagaatcaggggataacgcaggaaagaacatgtgagcaaaaggccagcaaaaggccaggaaccgtaaaaaggccgcgttgctggcgtttttccataggctccgcccccctgacgagcatcacaaaaatcgacgctcaagtcagaggtggcgaaacccgacaggactataaagataccaggcgtttccccctggaagctccctcgtgcgctctcctgttccgaccctgccgcttaccggatacctgtccgcctttctcccttcgggaagcgtggcgctttctcatagctcacgctgtaggtatctcagttcggtgtaggtcgttcgctccaagctgggctgtgtgcacgaaccccccgttcagcccgaccgctgcgccttatccggtaactatcgtcttgagtccaacccggtaagacacgacttatcgccactggcagcagccactggtaacaggattagcagagcgaggtatgtaggcggtgctacagagttcttgaagtggtggcctaactacggctacactagaagaacagtatttggtatctgcgctctgctgaagccagttaccttcggaaaaagagttggtagctcttgatccggcaaacaaaccaccgctggtagcggtggtttttttgtttgcaagcagcagattacgcgcagaaaaaaaggatctcaagaagatcctttgatcttttctacggggtctgacgctcagtggaacgaaaactcacgttaagggattttggtcatgagattatcaaaaaggatcttcacctagatccttttaaattaaaaatgaagttttaaatcaatctaaagtatatatgagtaaacttggtctgacagttaccaatgcttaatcagtgaggcacctatctcagcgatctgtctatttcgttcatccatagttgcctgactccccgtcgtgtagataactacgatacgggagggcttaccatctggccccagtgctgcaatgataccgcgagacccacgctcaccggctccagatttatcagcaataaaccagccagccggaagggccgagcgcagaagtggtcctgcaactttatccgcctccatccagtctattaattgttgccgggaagctagagtaagtagttcgccagttaatagtttgcgcaacgttgttgccattgctacaggcatcgtggtgtcacgctcgtcgtttggtatggcttcattcagctccggttcccaacgatcaaggcgagttacatgatcccccatgttgtgcaaaaaagcggttagctccttcggtcctccgatcgttgtcagaagtaagttggccgcagtgttatcactcatggttatggcagcactgcataattctcttactgtcatgccatccgtaagatgcttttctgtgactggtgagtactcaaccaagtcattctgagaatagtgtatgcggcgaccgagttgctcttgcccggcgtcaatacgggataataccgcgccacatagcagaactttaaaagtgctcatcattggaaaacgttcttcggggcgaaaactctcaaggatcttaccgctgttgagatccagttcgatgtaacccactcgtgcacccaactgatcttcagcatcttttactttcaccagcgtttctgggtgagcaaaaacaggaaggcaaaatgccgcaaaaaagggaataagggcgacacggaaatgttgaatactcatactcttcctttttcaatattattgaagcatttatcagggttattgtctcatgagcggatacatatttgaatgtatttagaaaaataaacaaataggggttccgcgcacatttccccgaaaagtgccacctgacgtcgacggatcgggagatctcccgatcccctatggtgcactctcagtacaatctgctctgatgccgcatagttaagccagtatctgctccctgcttgtgtgttggaggtcgctgagtagtgcgcgagcaaaatttaagctacaacaaggcaaggcttgaccgacaattgcatgaagaatctgcttagggttaggcgttttgcgctgcttcgcgatgtacgggccagatatacgcgttgacattgattattgactagttattaatagtaatcaattacggggtcattagttcatagcccatatatggagttccgcgttacataacttacggtaaatggcccgcctggctgaccgcccaacgacccccgcccattgacgtcaataatgacgtatgttcccatagtaacgccaatagggactttccattgacgtcaatgggtggagtatttacggtaaactgcccacttggcagtacatcaagtgtatcatatgccaagtacgccccctattgacgtcaatgacggtaaatggcccgcctggcattatgcccagtacatgaccttatgggactttcctacttggcagtacatctacgtattagtcatcgctattaccatggtgatgcggttttggcagtacatcaatgggcgtggatagcggtttgactcacggggatttccaagtctccaccccattgacgtcaatgggagtttgttttggcaccaaaatcaacgggactttccaaaatgtcgtaacaactccgccccattgacgcaaatgggcggtaggcgtgtacggtgggaggtctatataagcagcgcgttttgcctgtactgggtctctctggttagaccagatctgagcctgggagctctctggctaactagggaacccactgcttaagcctcaataaagcttgccttgagtgcttcaagtagtgtgtgcccgtctgttgtgtgactctggtaactagagatccctcagacccttttagtcagtgtggaaaatctctagcagtggcgcccgaacagggacttgaaagcgaaagggaaaccagaggagctctctcgacgcaggactcggcttgctgaagcgcgcacggcaagaggcgaggggcggcgactggtgagtacgccaaaaattttgactagcggaggctagaaggagagagatgggtgcgagagcgtcagtattaagcgggggagaattagatcgcgatgggaaaaaattcggttaaggccagggggaaagaaaaaatataaattaaaacatatagtatgggcaagcagggagctagaacgattcgcagttaatcctggcctgttagaaacatcagaaggctgtagacaaatactgggacagctacaaccatcccttcagacaggatcagaagaacttagatcattatataatacagtagcaaccctctattgtgtgcatcaaaggatagagataaaagacaccaaggaagctttagacaagatagaggaagagcaaaacaaaagtaagaccaccgcacagcaagcggccgctgatcttcagacctggaggaggagatatgagggacaattggagaagtgaattatataaatataaagtagtaaaaattgaaccattaggagtagcacccaccaaggcaaagagaagagtggtgcagagagaaaaaagagcagtgggaataggagctttgttccttgggttcttgggagcagcaggaagcactatgggcgcagcgtcaatgacgctgacggtacaggccagacaattattgtctggtatagtgcagcagcagaacaatttgctgagggctattgaggcgcaacagcatctgttgcaactcacagtctggggcatcaagcagctccaggcaagaatcctggctgtggaaagatacctaaaggatcaacagctcctggggatttggggttgctctggaaaactcatttgcaccactgctgtgccttggaatgctagttggagtaataaatctctggaacagatttggaatcacacgacctggatggagtgggacagagaaattaacaattacacaagcttaatacactccttaattgaagaatcgcaaaaccagcaagaaaagaatgaacaagaattattggaattagataaatgggcaagtttgtggaattggtttaacataacaaattggctgtggtatataaaattattcataatgatagtaggaggcttggtaggtttaagaatagtttttgctgtactttctatagtgaatagagttaggcagggatattcaccattatcgtttcagacccacctcccaaccccgaggggacccgacaggcccgaaggaatagaagaagaaggtggagagagagacagagacagatccattcgattagtgaacggatcggcactgcgtgcgccaattctgcagacaaatggcagtattcatccacaattttaaaagaaaaggggggattggggggtacagtgcaggggaaagaatagtagacataatagcaacagacatacaaactaaagaattacaaaaacaaattacaaaaattcaaaattttcgggtttattacagggacagcagagatccagtttggttaattaaggtaccgagggcctatttcccatgattccttcatatttgcatatacgatacaaggctgttagagagataattagaattaatttgactgtaaacacaaagatattagtacaaaatacgtgacgtagaaagtaataatttcttgggtagtttgcagttttaaaattatgttttaaaatggactatcatatgcttaccgtaacttgaaagtatttcgatttcttggctttatatatcttgtggaaaggacgaaacaccg

SEQ ID NO: 111 - DNA, 6733 bp, synthetic construct
  misc_feature 1..6733: note = reporter vector
  source 1..6733: mol_type = other DNA
aatcaacctctggattacaaaatttgtgaaagattgactggtattcttaactatgttgctccttttacgctatgtggatacgctgctttaatgcctttgtatcatgctattgcttcccgtatggctttcattttctcctccttgtataaatcctggttgctgtctctttatgaggagttgtggcccgttgtcaggcaacgtggcgtggtgtgcactgtgtttgctgacgcaacccccactggttggggcattgccaccacctgtcagctcctttccgggactttcgctttccccctccctattgccacggcggaactcatcgccgcctgccttgcccgctgctggacaggggctcggctgttgggcactgacaattccgtggtgttgtcggggaagctgacgtcctttccatggctgctcgcctgtgttgccacctggattctgcgcgggacgtccttctgctacgtcccttcggccctcaatccagcggaccttccttcccgcggcctgctgccggctctgcggcctcttccgcgtctccgccttcgccctcagacgagtcggatctccctttggccgcctccccgccaccggttaggggcccgtttaaacccgctgatcagcctcgactgtgccttctagttgccagccatctgttgtttgcccctcccccgtgccttccttgaccctggaaggtgccactcccactgtcctttcctaataaaatgaggaaattgcatcgcattgtctgagtaggtgtcattctattctggggggtggggtggggcaggacagcaagggggaggattgggaagacaatagcaggcatgctggggatgcggtgggctctatgggctcgagggggttggggttgcgccttttccaaggcagccctgggtttgcgcagggacgcggctgctctgggcgtggttccgggaaacgcagcggcgccgaccctgggactcgcacattcttcacgtccgttcgcagcgtcacccggatcttcgccgctacccttgtgggccccccggcgacgcttcctgctccgcccctaagtcgggaaggttccttgcggttcgcggcgtgccggacgtgacaaacggaagccgcacgtctcactagtaccctcgcagacggacagcgccagggagcaatggcagcgcgccgaccgcgatgggctgtggccaatagcggctgctcagcagggcgcgccgagagcagcggccgggaaggggcggtgcgggaggcggggtgtggggcggtagtgtgggccctgttcctgcccgcgcggtgttccgcattctgcaagcctccggagcgcacgtcggcagtcggctccctcgttgaccgaatcaccgacctctctccccagggggatccaccggagcttaccatgaccgagtacaagcccacggtgcgcctcgccacccgcgacgacgtccccagggccgtacgcaccctcgccgccgcgttcgccgactaccccgccacgcgccacaccgtcgatccggaccgccacatcgagcgggtcaccgagctgcaagaactcttcctcacgcgcgtcgggctcgacatcggcaaggtgtgggtcgcggacgacggcgccgcggtggcggtctggaccacgccggagagcgtcgaagcgggggcggtgttcgccgagatcggcccgcgcatggccgagttgagcggttcccggctggccgcgcagcaacagatggaaggcctcctggcgccgcaccggcccaaggagcccgcgtggttcctggccaccgtcggcgtctcgcccgaccaccagggcaagggtctgggcagcgccgtcgtgctccccggagtggaggcggccgagcgcgccggggtgcccgccttcctggaaacctccgcgccccgcaacctccccttctacgagcggctcggcttcaccgtcaccgccgacgtcgaggtgcccgaaggaccgcgcacctggtgcatgacccgcaagcccggtgcctgacgcccgccccacgacccgcagcgcccgaccgaaaggagcgcacgaccccatgcatcggtacctttaagaccaatgacttacaaggcagctgtagatcttagccactttctagagtcggggcggccggccgcttcgagcagacatgataagatacattgatgagtttggacaaaccacaactagaatgcagtgaaaaaaatgctttatttgtgaaatttgtgatgctattgctttatttgtaaccattataagctgcaataaacaagttaacatggcggcgcgcctaaaagttttgttactttatagaagaaattttgagtttttgtttttttttaataaataaataaacataaataaattgtttgttgaatttattattagtatgtaagtgtaaatataataaaacttaatatctattcaaattaataaataaacctcgatatacagaccgataaaacacatgcgtcaattttacgcatgattatctttaacgtacgtcacaatatgattatctttctagggttaaggccggccaaaagggcgaattctgcagatatccatcacactggcggccgctcgagcatgcatctagagggcccaattcgccctatagtgagtcgtattacaattcactggccgtcgttttacaacgtcgtgactgggaaaaccctggcgttacccaacttaatcgccttgcagcacatccccctttcgccagctggcgtaatagcgaagaggcccgcaccgatcgcccttcccaacagttgcgcagcctgaatggcgaatggacgcgccctgtagcggcgcattaagcgcggcgggtgtggtggttacgcgcagcgtgaccgctacacttgccagcgccctagcgcccgctcctttcgctttcttcccttcctttctcgccacgttcgccggctttccccgtcaagctctaaatcgggggctccctttagggttccgatttagtgctttacggcacctcgaccccaaaaaacttgattagggtgatggttcacgtagtgggccatcgccctgatagacggtttttcgccctttgacgttggagtccacgttctttaatagtggactcttgttccaaactggaacaacactcaaccctatctcggtctattcttttgatttataagggattttgccgatttcggcctattggttaaaaaatgagctgatttaacaaaaatttaacgcgaattttaacaaaattcagggcgcaagggctgctaaaggaagcggaacacgtagaaagccagtccgcagaaacggtgctgaccccggatgaatgtcagctactgggctatctggacaagggaaaacgcaagcgcaaagagaaagcaggtagcttgcagtgggcttacatggcgatagctagactgggcggttttatggacagcaagcgaaccggaattgccagctggggcgccctctggtaaggttgggaagccctgcaaagtaaactggatggctttcttgccgccaaggatctgatggcgcaggggatcaagatctgatcaagagacaggatgaggatcgtttcgcatgattgaacaagatggattgcacgcaggttctccggccgcttgggtggagaggctattcggctatgactgggcacaacagacaatcggctgctctgatgccgccgtgttccggctgtcagcgcaggggcgcccggttctttttgtcaagaccgacctgtccggtgccctgaatgaactgcaggacgaggcagcgcggctatcgtggctggccacgacgggcgttccttgcgcagctgtgctcgacgttgtcactgaagcgggaagggactggctgctattgggcgaagtgccggggcaggatctcctgtcatcccaccttgctcctgccgagaaagtatccatcatggctgatgcaatgcggcggctgcatacgcttgatccggctacctgcccattcgaccaccaagcgaaacatcgcatcgagcgagcacgtactcggatggaagccggtcttgtcgatcaggatgatctggacgaagagcatcaggggctcgcgccagccgaactgttcgccaggctcaaggcgcgcatgcccgacggcgaggatctcgtcgtgacccatggcgatgcctgcttgccgaatatcatggtggaaaatggccgcttttctggattcatcgactgtggccggctgggtgtggcggaccgctatcaggacatagcgttggctacccgtgatattgctgaagagcttggcggcgaatgggctgaccgcttcctcgtgctttacggtatcgccgctcccgattcgcagcgcatcgccttctatcgccttcttgacgagttcttctgaattgaaaaaggaagagtatgagtattcaacatttccgtgtcgcccttattcccttttttgcggcattttgccttcctgtttttgctcacccagaaacgctggtgaaagtaaaagatgctgaagatcagttgggtgcacgagtgggttacatcgaactggatctcaacagcggtaagatccttgagagttttcgccccgaagaacgttttccaatgatgagcacttttaaagttctgctatgtggcgcggtattatcccgtattgacgccgggcaagagcaactcggtcgccgcatacactattctcagaatgacttggttgagtactcaccagtcacagaaaagcatcttacggatggcatgacagtaagagaattatgcagtgctgccataaccatgagtgataacactgcggccaacttacttctgacaacgatcggaggaccgaaggagctaaccgcttttttgcacaacatgggggatcatgtaactcgccttgatcgttgggaaccggagctgaatgaagccataccaaacgacgagcgtgacaccacgatgcctgtagcaatggcaacaacgttgcgcaaactattaactggcgaactacttactctagcttcccggcaacaattaatagactggatggaggcggataaagttgcaggaccacttctgcgctcggcccttccggctggctggtttattgctgataaatctggagccggtgagcgtgggtctcgcggtatcattgcagcactggggccagatggtaagccctcccgtatcgtagttatctacacgacggggagtcaggcaactatggatgaacgaaatagacagatcgctgagataggtgcctcactgattaagcattggtaactgtcagaccaagtttactcatatatactttagattgatttaaaacttcatttttaatttaaaaggatctaggtgaagatcctttttgataatctcatgaccaaaatcccttaacgtgagttttcgttccactgagcgtcagaccccgtagaaaagatcaaaggatcttcttgagatcctttttttctgcgcgtaatctgctgcttgcaaacaaaaaaaccaccgctaccagcggtggtttgtttgccggatcaagagctaccaactctttttccgaaggtaactggcttcagcagagcgcagataccaaatactgttcttctagtgtagccgtagttaggccaccacttcaagaactctgtagcaccgcctacatacctcgctctgctaatcctgttaccagtggctgctgccagtggcgataagtcgtgtcttaccgggttggactcaagacgatagttaccggataaggcgcagcggtcgggctgaacggggggttcgtgcacacagcccagcttggagcgaacgacctacaccgaactgagatacctacagcgtgagctatgagaaagcgccacgcttcccgaagggagaaaggcggacaggtatccggtaagcggcagggtcggaacaggagagcgcacgagggagcttccagggggaaacgcctggtatctttatagtcctgtcgggtttcgccacctctgacttgagcgtcgatttttgtgatgctcgtcaggggggcggagcctatggaaaaacgccagcaacgcggcctttttacggttcctggccttttgctggccttttgctcacatgttctttcctgcgttatcccctgattctgtggataaccgtattaccgcctttgagtgagctgataccgctcgccgcagccgaacgaccgagcgcagcgagtcagtgagcgaggaagcggaagagcgcccaatacgcaaaccgcctctccccgcgcgttggccgattcattaatgcagctggcacgacaggtttcccgactggaaagcgggcagtgagcgcaacgcaattaatgtgagttagctcactcattaggcaccccaggctttacactttatgcttccggctcgtatgttgtgtggaattgtgagcggataacaatttcacacaggaaacagctatgaccatgattacgccaagcttggtaccttaaccctagaaagatagtctgcgtaaaattgacgcatgcattcttgaaatattgctctctctttctaaatagcgcgaatccgtcgctgtgcatttaggacatctcagtcgccgcttggagctcccgtgaggcgtgcttgtcaatgcggtaagtgtcactgattttgaactataacgaccgcgtgagtcaaaatgacgcatgattatcttttacgtgacttttaagatttaactcatacgataattatattgttatttcatgttctacttacgtgataacttattatatatatattttcttgttatagatatcattaattaa

SEQ ID NO: 112 - RNA, 20 nt, synthetic construct
  modified_base 3: mod_base = OTHER; note = thymine
  modified_base 12: mod_base = OTHER; note = thymine
  modified_base 15: mod_base = OTHER; note = thymine
  misc_feature 1..20: note = EGFP gRNA
  source 1..20: mol_type = other RNA
catgccgagagtgatcccgg

SEQ ID NO: 113 - RNA, 20 nt, synthetic construct
  misc_feature 1..20: note = NT gRNA
  source 1..20: mol_type = other RNA
  modified_base 6: mod_base = OTHER; note = thymine
  modified_base 11: mod_base = OTHER; note = thymine
  modified_base 13: mod_base = OTHER; note = thymine
cccgatcaggtataccgaac